European Patent Application EP 4 316 514 A1, published February 7, 2024. Title: MVA-BASED VECTORS AND THEIR USE AS VACCINE AGAINST SARS-CoV-2. Applicant: CONSEJO SUPERIOR DE INVESTIGACIONES CIENTIFICAS. The sequence listing filed with the application follows.

SEQUENCE LISTING (28 sequences)

SEQ ID NO: 1 - DNA, 3822 bp, synthetic construct
  misc_feature 1..3822: note = Nucleic acid encoding for the S protein from MVA-S
  source 1..3822: mol_type = other DNA
atgtttgtatttttagtattattaccattagtatcttctcaatgtgtaaatttaactactagaactcaattgccaccagcttatactaattcttttactagaggagtatattatccagataaagtatttagatcttctgtattacattctactcaagatttatttttaccatttttttctaatgtaacttggtttcatgctatacatgtatctggaactaatggaactaaaagatttgataatccagtattaccatttaatgatggagtatattttgcttctactgaaaaatctaatataataagaggatggatatttggaactactttagattctaaaactcaatctttattaatagtaaataatgctactaatgtagtaataaaagtatgtgaatttcaattttgtaatgatccatttttaggagtatattatcataaaaataataaatcttggatggaatctgaatttagagtatattcttctgctaataattgtacttttgaatatgtatctcaaccatttttaatggatttagaaggaaaacaaggaaattttaaaaatttaagagaatttgtatttaaaaatatagatggatattttaaaatatattctaaacatactccaataaatttagtaagagatttaccacaaggattttctgctttagaaccattagtagatttaccaataggaataaatataactagatttcaaactttattagctttacatagatcttatttaactccaggagattcttcttctggatggactgctggagctgctgcttattatgtaggatatttacaaccaagaacttttttattaaaatataatgaaaatggaactataactgatgctgtagattgtgctttagatccattatctgaaactaaatgtactttaaaatcttttactgtagaaaaaggaatatatcaaacttctaattttagagtacaaccaactgaatctatagtaagatttccaaatataactaatttatgtccatttggagaagtatttaatgctactagatttgcttctgtatatgcttggaatagaaaaagaatatctaattgtgtagctgattattctgtattatataattctgcttctttttctacttttaaatgttatggagtatctccaactaaattaaatgatttatgttttactaatgtatatgctgattcttttgtaataagaggagatgaagtaagacaaatagctccaggacaaactggaaaaatagctgattataattataaattaccagatgattttactggatgtgtaatagcttggaatagtaataatttagattctaaagtaggaggaaattataattatttatatagattatttagaaaatctaatttaaaaccatttgaaagagatatatctactgaaatatatcaagctggatctactccatgtaatggagtagaaggatttaattgttattttccattacaatcttatggatttcaaccaactaatggagtaggatatcaaccatatagagtagtagtattatcttttgaattattacatgctccagctactgtatgtggaccaaaaaaatctactaatttagtaaaaaataaatgtgtaaattttaattttaatggattaactggaactggagtattaactgaatctaataaaaaatttttaccatttcaacaatttggaagagatatagctgatactactgatgctgtaagagatccacaaactttagaaatattagatataactccatgttcttttggaggagtatctgtaataactccaggaactaatacttctaatcaagtagctgtattatatcaagatgtaaattgtactgaagtaccagtagctatacatgctgatcaattaactccaacttggagagtatattctactggatctaatgtatttcaaactagagctggatgtttaataggagctgaacatgtaaataattcttatgaatgtgatataccaataggagctggaatatgtgcttcttatcaaactcaaactaattctccaagaagagctagatctgtagctagccaatctataatagcttatactatgtctttaggagctgaaaattctgtagcttattctaataattctatagctataccaactaattttactatatctgtaactactgaaatattaccagtatctatgactaaaacttctgtagattgtactatgtatatatgtggagattctactgaatgttctaatttattattacaatatggatctttttgtactcaattaaatagagctttaactggaatagctgtagaacaagataaaaatactcaagaagtatttgctcaagtaaaacaaatatataaaactccaccaataaaagattttggaggatttaatttttctcaaatattaccagatccatctaaaccatctaaaagatcttttatagaagatttattatttaataaagtaactttagctgatgctggatttataaaacaatatggagattgtttaggagatatagctgctagagatttaatatgtgctcaaaaatttaatggattaactgtattaccaccattattaactgatgaaatgatagctcaatatacttctgctttattagctggaactataacttctggatggacttttggagctggagctgctttacaaataccatttgctatgcaaatggcttatagatttaatggaataggagtaactcaaaatgtattatatgaaaatcaaaaattaatagctaatcaatttaattctgctataggaaaaatacaagattctttatcttctactgcttctgctttaggaaaattacaagatgtagtaaatcaaaatgctcaagcattaaatactttagtaaaacaattatcttctaattttggagctatatcttctgtattaaatgatatattatctagattagataaagtagaagctgaagtacaaatagatagattaataactggaagattacaatctttacaaacttatgtaactcaacaattaataagagctgctgaaataagagcttctgctaatttagctgctactaaaatgtctgaatgtgtattaggacaatctaaaagagtagatttttgtggaaaaggatatcatttaatgtcttttccacaatctgctccacatggagtagtatttttacatgtaacttatgtaccagctcaagaaaaaaattttactactgctccagctatatgtcatgatggaaaagctcattttccaagagaaggagtatttgtatctaatggaactcattggtttgtaactcaaagaaatttttatgaaccacaaataataactactgataatacttttgtatctggaaattgtgatgtagtaataggaatagtaaataatactgtatatgatccattacaaccagaattagattcttttaaagaagaattagataaatattttaaaaatcatacttctccagatgtagatttaggagatatatctggaataaatgcttctgtagtaaatatacaaaaagaaatagatagattaaatgaagtagctaaaaatttaaatgaatctttaatagatttacaagaattaggaaaatatgaacaatatataaaatggccatggtatatatggttaggatttatagctggattaatagctatagtaatggtaactataatgttatgttgtatgacttcttgttgttcttgtttaaaaggatgttgttcttgtggatcttgttgtaaatttgatgaagatgattctgaaccagtattaaaaggagtaaaattacattatacttaa

SEQ ID NO: 2 - protein, 1273 aa, synthetic construct
  REGION 1..1273: note = Amino acid sequence of S protein from MVA-S also represented inFig. 20
MFVFLVLLPLVSSQCVNLTTRTQLPPAYTNSFTRGVYYPDKVFRSSVLHSTQDLFLPFFSNVTWFHAIHVSGTNGTKRFDNPVLPFNDGVYFASTEKSNIIRGWIFGTTLDSKTQSLLIVNNATNVVIKVCEFQFCNDPFLGVYYHKNNKSWMESEFRVYSSANNCTFEYVSQPFLMDLEGKQGNFKNLREFVFKNIDGYFKIYSKHTPINLVRDLPQGFSALEPLVDLPIGINITRFQTLLALHRSYLTPGDSSSGWTAGAAAYYVGYLQPRTFLLKYNENGTITDAVDCALDPLSETKCTLKSFTVEKGIYQTSNFRVQPTESIVRFPNITNLCPFGEVFNATRFASVYAWNRKRISNCVADYSVLYNSASFSTFKCYGVSPTKLNDLCFTNVYADSFVIRGDEVRQIAPGQTGKIADYNYKLPDDFTGCVIAWNSNNLDSKVGGNYNYLYRLFRKSNLKPFERDISTEIYQAGSTPCNGVEGFNCYFPLQSYGFQPTNGVGYQPYRVVVLSFELLHAPATVCGPKKSTNLVKNKCVNFNFNGLTGTGVLTESNKKFLPFQQFGRDIADTTDAVRDPQTLEILDITPCSFGGVSVITPGTNTSNQVAVLYQDVNCTEVPVAIHADQLTPTWRVYSTGSNVFQTRAGCLIGAEHVNNSYECDIPIGAGICASYQTQTNSPRRARSVASQSIIAYTMSLGAENSVAYSNNSIAIPTNFTISVTTEILPVSMTKTSVDCTMYICGDSTECSNLLLQYGSFCTQLNRALTGIAVEQDKNTQEVFAQVKQIYKTPPIKDFGGFNFSQILPDPSKPSKRSFIEDLLFNKVTLADAGFIKQYGDCLGDIAARDLICAQKFNGLTVLPPLLTDEMIAQYTSALLAGTITSGWTFGAGAALQIPFAMQMAYRFNGIGVTQNVLYENQKLIANQFNSAIGKIQDSLSSTASALGKLQDVVNQNAQALNTLVKQLSSNFGAISSVLNDILSRLDKVEAEVQIDRLITGRLQSLQTYVTQQLIRAAEIRASANLAATKMSECVLGQSKRVDFCGKGYHLMSFPQSAPHGVVFLHVTYVPAQEKNFTTAPAICHDGKAHFPREGVFVSNGTHWFVTQRNFYEPQIITTDNTFVSGNCDVVIGIVNNTVYDPLQPELDSFKEELDKYFKNHTSPDVDLGDISGINASVVNIQKEIDRLNEVAKNLNESLIDLQELGKYEQYIKWPWYIWLGFIAGLIAIVMVTIMLCCMTSCCSCLKGCCSCGSCCKFDEDDSEPVLKGVKLHYT

SEQ ID NO: 3 - DNA, 3822 bp, synthetic construct
  misc_feature 1..3822: note = Nucleic acid encoding for the S protein from MVA-Sdg
  source 1..3822: mol_type = other DNA
atgtttgtatttttagtattattaccattagtatcttctcaatgtgtaaatttaactactagaactcaattgccaccagcttatactaattcttttactagaggagtatattatccagataaagtatttagatcttctgtattacattctactcaagatttatttttaccatttttttctaatgtaacttggtttcatgctatacatgtatctggaactaatggaactaaaagatttgataatccagtattaccatttaatgatggagtatattttgcttctactgaaaaatctaatataataagaggatggatatttggaactactttagattctaaaactcaatctttattaatagtaaataatgctactaatgtagtaataaaagtatgtgaatttcaattttgtaatgatccatttttaggagtatattatcataaaaataataaatcttggatggaatctgaatttagagtatattcttctgctaataattgtacttttgaatatgtatctcaaccatttttaatggatttagaaggaaaacaaggaaattttaaaaatttaagagaatttgtatttaaaaatatagatggatattttaaaatatattctaaacatactccaataaatttagtaagagatttaccacaaggattttctgctttagaaccattagtagatttaccaataggaataaatataactagatttcaaactttattagctttacatagatcttatttaactccaggagattcttcttctggatggactgctggagctgctgcttattatgtaggatatttacaaccaagaacttttttattaaaatataatgaaaatggaactataactgatgctgtagattgtgctttagatccattatctgaaactaaatgtactttaaaatcttttactgtagaaaaaggaatatatcaaacttctaattttagagtacaaccaactgaatctatagtaagatttccaaatataactaatttatgtccatttggagaagtatttaatgctactagatttgcttctgtatatgcttggaatagaaaaagaatatctaattgtgtagctgattattctgtattatataattctgcttctttttctacttttaaatgttatggagtatctccaactaaattaaatgatttatgttttactaatgtatatgctgattcttttgtaataagaggagatgaagtaagacaaatagctccaggacaaactggaaaaatagctgattataattataaattaccagatgattttactggatgtgtaatagcttggaatagtaataatttagattctaaagtaggaggaaattataattatttatatagattatttagaaaatctaatttaaaaccatttgaaagagatatatctactgaaatatatcaagctggatctactccatgtaatggagtagaaggatttaattgttattttccattacaatcttatggatttcaaccaactaatggagtaggatatcaaccatatagagtagtagtattatcttttgaattattacatgctccagctactgtatgtggaccaaaaaaatctactaatttagtaaaaaataaatgtgtaaattttaattttaatggattaactggaactggagtattaactgaatctaataaaaaatttttaccatttcaacaatttggaagagatatagctgatactactgatgctgtaagagatccacaaactttagaaatattagatataactccatgttcttttggaggagtatctgtaataactccaggaactaatacttctaatcaagtagctgtattatatcaaggagtaaattgtactgaagtaccagtagctatacatgctgatcaattaactccaacttggagagtatattctactggatctaatgtatttcaaactagagctggatgtttaataggagctgaacatgtaaataattcttatgaatgtgatataccaataggagctggaatatgtgcttcttatcaaactcaaactaattctccaagaagagctagatctgtagctagccaatctataatagcttatactatgtctttaggagctgaaaattctgtagcttattctaataattctatagctataccaactaattttactatatctgtaactactgaaatattaccagtatctatgactaaaacttctgtagattgtactatgtatatatgtggagattctactgaatgttctaatttattattacaatatggatctttttgtactcaattaaatagagctttaactggaatagctgtagaacaagataaaaatactcaagaagtatttgctcaagtaaaacaaatatataaaactccaccaataaaagattttggaggatttaatttttctcaaatattaccagatccatctaaaccatctaaaagatcttttatagaagatttattatttaataaagtaactttagctgatgctggatttataaaacaatatggagattgtttaggagatatagctgctagagatttaatatgtgctcaaaaatttaatggattaactgtattaccaccattattaactgatgaaatgatagctcaatatacttctgctttattagctggaactataacttctggatggacttttggagctggagctgctttacaaataccatttgctatgcaaatggcttatagatttaatggaataggagtaactcaaaatgtattatatgaaaatcaaaaattaatagctaatcaatttaattctgctataggaaaaatacaagattctttatcttctactgcttctgctttaggaaaattacaagatgtagtaaatcaaaatgctcaagcattaaatactttagtaaaacaattatcttctaattttggagctatatcttctgtattaaatgatatattatctagattagataaagtagaagctgaagtacaaatagatagattaataactggaagattacaatctttacaaacttatgtaactcaacaattaataagagctgctgaaataagagcttctgctaatttagctgctactaaaatgtctgaatgtgtattaggacaatctaaaagagtagatttttgtggaaaaggatatcatttaatgtcttttccacaatctgctccacatggagtagtatttttacatgtaacttatgtaccagctcaagaaaaaaattttactactgctccagctatatgtcatgatggaaaagctcattttccaagagaaggagtatttgtatctaatggaactcattggtttgtaactcaaagaaatttttatgaaccacaaataataactactgataatacttttgtatctggaaattgtgatgtagtaataggaatagtaaataatactgtatatgatccattacaaccagaattagattcttttaaagaagaattagataaatattttaaaaatcatacttctccagatgtagatttaggagatatatctggaataaatgcttctgtagtaaatatacaaaaagaaatagatagattaaatgaagtagctaaaaatttaaatgaatctttaatagatttacaagaattaggaaaatatgaacaatatataaaatggccatggtatatatggttaggatttatagctggattaatagctatagtaatggtaactataatgttatgttgtatgacttcttgttgttcttgtttaaaaggatgttgttcttgtggatcttgttgtaaatttgatgaagatgattctgaaccagtattaaaaggagtaaaattacattatacttaa

SEQ ID NO: 4 - protein, 1273 aa, synthetic construct
  REGION 1..1273: note = Amino acid sequence of S protein from MVA-Sdg also represented inFig. 20
MFVFLVLLPLVSSQCVNLTTRTQLPPAYTNSFTRGVYYPDKVFRSSVLHSTQDLFLPFFSNVTWFHAIHVSGTNGTKRFDNPVLPFNDGVYFASTEKSNIIRGWIFGTTLDSKTQSLLIVNNATNVVIKVCEFQFCNDPFLGVYYHKNNKSWMESEFRVYSSANNCTFEYVSQPFLMDLEGKQGNFKNLREFVFKNIDGYFKIYSKHTPINLVRDLPQGFSALEPLVDLPIGINITRFQTLLALHRSYLTPGDSSSGWTAGAAAYYVGYLQPRTFLLKYNENGTITDAVDCALDPLSETKCTLKSFTVEKGIYQTSNFRVQPTESIVRFPNITNLCPFGEVFNATRFASVYAWNRKRISNCVADYSVLYNSASFSTFKCYGVSPTKLNDLCFTNVYADSFVIRGDEVRQIAPGQTGKIADYNYKLPDDFTGCVIAWNSNNLDSKVGGNYNYLYRLFRKSNLKPFERDISTEIYQAGSTPCNGVEGFNCYFPLQSYGFQPTNGVGYQPYRVVVLSFELLHAPATVCGPKKSTNLVKNKCVNFNFNGLTGTGVLTESNKKFLPFQQFGRDIADTTDAVRDPQTLEILDITPCSFGGVSVITPGTNTSNQVAVLYQGVNCTEVPVAIHADQLTPTWRVYSTGSNVFQTRAGCLIGAEHVNNSYECDIPIGAGICASYQTQTNSPRRARSVASQSIIAYTMSLGAENSVAYSNNSIAIPTNFTISVTTEILPVSMTKTSVDCTMYICGDSTECSNLLLQYGSFCTQLNRALTGIAVEQDKNTQEVFAQVKQIYKTPPIKDFGGFNFSQILPDPSKPSKRSFIEDLLFNKVTLADAGFIKQYGDCLGDIAARDLICAQKFNGLTVLPPLLTDEMIAQYTSALLAGTITSGWTFGAGAALQIPFAMQMAYRFNGIGVTQNVLYENQKLIANQFNSAIGKIQDSLSSTASALGKLQDVVNQNAQALNTLVKQLSSNFGAISSVLNDILSRLDKVEAEVQIDRLITGRLQSLQTYVTQQLIRAAEIRASANLAATKMSECVLGQSKRVDFCGKGYHLMSFPQSAPHGVVFLHVTYVPAQEKNFTTAPAICHDGKAHFPREGVFVSNGTHWFVTQRNFYEPQIITTDNTFVSGNCDVVIGIVNNTVYDPLQPELDSFKEELDKYFKNHTSPDVDLGDISGINASVVNIQKEIDRLNEVAKNLNESLIDLQELGKYEQYIKWPWYIWLGFIAGLIAIVMVTIMLCCMTSCCSCLKGCCSCGSCCKFDEDDSEPVLKGVKLHYT

SEQ ID NO: 5 - protein, 1273 aa, synthetic construct
  REGION 1..1273: note = Amino acid sequence of S protein from MVA- Spfx and MVA-Spf andfig. 20
MFVFLVLLPLVSSQCVNLTTRTQLPPAYTNSFTRGVYYPDKVFRSSVLHSTQDLFLPFFSNVTWFHAIHVSGTNGTKRFDNPVLPFNDGVYFASTEKSNIIRGWIFGTTLDSKTQSLLIVNNATNVVIKVCEFQFCNDPFLGVYYHKNNKSWMESEFRVYSSANNCTFEYVSQPFLMDLEGKQGNFKNLREFVFKNIDGYFKIYSKHTPINLVRDLPQGFSALEPLVDLPIGINITRFQTLLALHRSYLTPGDSSSGWTAGAAAYYVGYLQPRTFLLKYNENGTITDAVDCALDPLSETKCTLKSFTVEKGIYQTSNFRVQPTESIVRFPNITNLCPFGEVFNATRFASVYAWNRKRISNCVADYSVLYNSASFSTFKCYGVSPTKLNDLCFTNVYADSFVIRGDEVRQIAPGQTGKIADYNYKLPDDFTGCVIAWNSNNLDSKVGGNYNYLYRLFRKSNLKPFERDISTEIYQAGSTPCNGVEGFNCYFPLQSYGFQPTNGVGYQPYRVVVLSFELLHAPATVCGPKKSTNLVKNKCVNFNFNGLTGTGVLTESNKKFLPFQQFGRDIADTTDAVRDPQTLEILDITPCSFGGVSVITPGTNTSNQVAVLYQGVNCTEVPVAIHADQLTPTWRVYSTGSNVFQTRAGCLIGAEHVNNSYECDIPIGAGICASYQTQTNSPSRASSVASQSIIAYTMSLGAENSVAYSNNSIAIPTNFTISVTTEILPVSMTKTSVDCTMYICGDSTECSNLLLQYGSFCTQLNRALTGIAVEQDKNTQEVFAQVKQIYKTPPIKDFGGFNFSQILPDPSKPSKRSFIEDLLFNKVTLADAGFIKQYGDCLGDIAARDLICAQKFNGLTVLPPLLTDEMIAQYTSALLAGTITSGWTFGAGAALQIPFAMQMAYRFNGIGVTQNVLYENQKLIANQFNSAIGKIQDSLSSTASALGKLQDVVNQNAQALNTLVKQLSSNFGAISSVLNDILSRLDPPEAEVQIDRLITGRLQSLQTYVTQQLIRAAEIRASANLAATKMSECVLGQSKRVDFCGKGYHLMSFPQSAPHGVVFLHVTYVPAQEKNFTTAPAICHDGKAHFPREGVFVSNGTHWFVTQRNFYEPQIITTDNTFVSGNCDVVIGIVNNTVYDPLQPELDSFKEELDKYFKNHTSPDVDLGDISGINASVVNIQKEIDRLNEVAKNLNESLIDLQELGKYEQYIKWPWYIWLGFIAGLIAIVMVTIMLCCMTSCCSCLKGCCSCGSCCKFDEDDSEPVLKGVKLHYT

SEQ ID NO: 6 - DNA, 3822 bp, synthetic construct
  misc_feature 1..3822: note = Nucleic acid encoding for the S protein from MVA-Spfx
  source 1..3822: mol_type = other DNA
atgtttgtatttttagtattattaccattagtatcttctcaatgtgtaaatttaactactagaactcaattgcccccggcctatactaattcgtttactcgtggtgtttactatcctgataaagtgtttcgatcgtctgtgcttcattcgactcaagatctatttttgcccttctttagtaatgttacatggttccatgctatacatgtatcgggtacaaacggtacgaagcgtttcgacaacccagtcttaccattcaatgacggagtttattttgccagtaccgagaaatcaaatatcatcagaggatggatttttggtactactttggatagtaagactcagtctctattaatcgtcaataacgcaacgaacgttgtaatcaaagtatgcgagtttcaattctgcaacgatccatttctaggtgtttactaccacaagaacaataagtcgtggatggaaagtgagttccgtgtgtactcttctgccaataactgcactttcgaatatgtttcacagccgtttttaatggacttagagggtaaacaaggtaatttcaaaaacttgagagaatttgtcttcaaaaatattgatggttatttcaaaatatattcaaagcatacgcccattaatcttgttcgagacctaccgcaaggtttttccgcattagaacccttagttgatctacccattggaatcaacattacaagattccagacattgttagctttacaccgttcgtatcttacacccggtgattcgtcatcaggatggaccgctggagctgctgcctattatgtcggttacttgcaaccgcgtacattcctattgaagtacaatgaaaatggaactattacagacgccgtggactgtgccttggatcctttatctgaaactaagtgtacattaaaatcttttacagtagaaaaaggtatttaccaaacgtccaacttccgtgtccaacccacggaatcgatagttagatttccgaatattacgaacctatgcccatttggagaagtctttaacgccacgcgttttgcctcagtttacgcttggaatcgtaagcgtattagtaactgcgtagcggattattccgtactatacaattccgcgtccttttcgactttcaaatgttacggagtgtcgcccactaaacttaacgatctttgtttcaccaacgtgtacgcagactcatttgtaatcagaggagacgaagtgcgacaaattgcgcctggtcagaccggaaaaatcgcagattacaattataaacttccggacgatttcactggttgtgtcattgcatggaattccaacaacctagacagtaaagtaggaggtaactataattacctatatagattattccgaaaatcaaatttaaaaccatttgaacgtgacatcagtacagagatataccaagcgggatctacgccgtgcaacggagtagagggatttaattgctatttcccgttacaatcgtacggattccaacccacgaacggagtaggttaccaaccgtaccgtgtcgtggtccttagttttgagttgttgcacgcacctgccaccgtgtgcggtcccaaaaagtcaacaaacttagtcaaaaacaaatgtgtcaacttcaattttaatggactaacaggaaccggagtcttgactgaatcaaacaaaaaattccttcctttccaacaattcggtcgtgatattgcggatacgacagatgcggtacgagacccgcaaacacttgagatattggatataaccccttgctcattcggtggtgtttcggtaatcacccctggaacaaacacgagtaaccaggtagccgtactttaccagggtgtgaactgtacagaggtgccagtcgcgatacatgcggatcagctaacgccaacgtggagagtatattctaccggaagtaatgtgttccaaaccagagccggatgtcttatcggtgcagaacatgtaaacaatagttacgagtgtgatatccccattggagcgggtatttgcgcaagttatcaaacccaaacaaactctccctctagagcctctagtgttgcctctcagagtatcattgcttacacgatgtcgttgggagcagaaaattctgttgcatattctaacaattcgatagcaattccaaccaatttcacgatatccgtaaccaccgagatcttgccagttagtatgactaaaacatcggttgactgcacaatgtatatatgcggtgattctactgagtgttcaaacttgcttcttcagtatggttcgttttgtactcagctaaatcgagccttgacgggaatagccgttgaacaagacaaaaatacgcaggaggtgtttgctcaagtcaaacaaatttacaagaccccacctatcaaggatttcggtggttttaacttttcccaaatattaccagacccatcaaagccaagtaagagatccttcatagaggacctattgtttaataaggtaacgttggcggacgcgggttttattaagcaatacggtgactgcttaggtgatatagctgccagagacttaatctgcgctcagaaattcaacggattaaccgttttaccaccattattgacggacgagatgatcgcgcagtatacctcggctttgctagctggtacgattacatccggttggactttcggtgccggtgcagccctacagataccatttgcgatgcaaatggcctatcgttttaatggaatcggtgtcacccagaacgtgctttacgagaaccagaagttaattgctaatcaattcaactctgcaatcggaaagattcaagactcattatctagtacagcctccgccttaggaaagttacaggacgttgtgaaccagaatgctcaggcgttaaataccttggtcaaacaactatcctcaaatttcggtgcgatatcttcagtcttgaatgatatcctaagtcgactagatccacctgaggctgaagtacagattgaccgacttatcacaggtcgtctacaaagtttgcagacgtatgtgacccaacagctaataagagcggctgagatacgtgcttctgccaatttagcagctacaaaaatgtcagagtgtgtgctaggacaatcgaaacgagttgacttctgtggaaagggttaccacttgatgtcattcccccaaagtgcgcctcatggtgtggttttcttgcatgtaacgtacgtacccgcgcaagaaaagaattttactaccgccccggccatttgtcatgacggaaaagctcattttccgcgtgaaggtgtattcgtatccaacggtacgcactggtttgtgacccaaagaaacttttatgaaccgcagattataacgaccgacaatacgttcgtgtctggaaattgcgacgttgtaattggaatcgtaaacaatacagtttacgacccattgcaacccgagctagatagttttaaggaagaacttgacaagtattttaagaaccacacgtcaccggacgtcgacttgggagatatttcgggaattaacgctagtgttgtgaatatccagaaagaaatagatcgactaaatgaagtggccaagaaccttaacgagtccctaattgacttacaggaattgggtaagtatgaacaatacataaaatggccatggtatatatggttaggatttatagctggattaatagctatagtaatggttactatcatgttatgctgcatgacctcctgctgttcatgtttaaaaggatgttgctcctgcggttcgtgttgtaagttcgatgaagatgactccgaacctgtcttgaagggagtgaaattgcattacacttaa

SEQ ID NO: 7 - DNA, 3822 bp, synthetic construct
  misc_feature 1..3822: note = Nucleic acid encoding for the S protein from MVA-Spf
  source 1..3822: mol_type = other DNA
atgtttgtatttttagtattattaccattagtatcttctcaatgtgtaaatttaactactagaactcaattgccaccagcttatactaattcttttactagaggagtatattatccagataaagtatttagatcttctgtattacattctactcaagatttatttttaccatttttttctaatgtaacttggtttcatgctatacatgtatctggaactaatggaactaaaagatttgataatccagtattaccatttaatgatggagtatattttgcttctactgaaaaatctaatataataagaggatggatatttggaactactttagattctaaaactcaatctttattaatagtaaataatgctactaatgtagtaataaaagtatgtgaatttcaattttgtaatgatccatttttaggagtatattatcataaaaataataaatcttggatggaatctgaatttagagtatattcttctgctaataattgtacttttgaatatgtatctcaaccatttttaatggatttagaaggaaaacaaggaaattttaaaaatttaagagaatttgtatttaaaaatatagatggatattttaaaatatattctaaacatactccaataaatttagtaagagatttaccacaaggattttctgctttagaaccattagtagatttaccaataggaataaatataactagatttcaaactttattagctttacatagatcttatttaactccaggagattcttcttctggatggactgctggagctgctgcttattatgtaggatatttacaaccaagaacttttttattaaaatataatgaaaatggaactataactgatgctgtagattgtgctttagatccattatctgaaactaaatgtactttaaaatcttttactgtagaaaaaggaatatatcaaacttctaattttagagtacaaccaactgaatctatagtaagatttccaaatataactaatttatgtccatttggagaagtatttaatgctactagatttgcttctgtatatgcttggaatagaaaaagaatatctaattgtgtagctgattattctgtattatataattctgcttctttttctacttttaaatgttatggagtatctccaactaaattaaatgatttatgttttactaatgtatatgctgattcttttgtaataagaggagatgaagtaagacaaatagctccaggacaaactggaaaaatagctgattataattataaattaccagatgattttactggatgtgtaatagcttggaatagtaataatttagattctaaagtaggaggaaattataattatttatatagattatttagaaaatctaatttaaaaccatttgaaagagatatatctactgaaatatatcaagctggatctactccatgtaatggagtagaaggatttaattgttattttccattacaatcttatggatttcaaccaactaatggagtaggatatcaaccatatagagtagtagtattatcttttgaattattacatgctccagctactgtatgtggaccaaaaaaatctactaatttagtaaaaaataaatgtgtaaattttaattttaatggattaactggaactggagtattaactgaatctaataaaaaatttttaccatttcaacaatttggaagagatatagctgatactactgatgctgtaagagatccacaaactttagaaatattagatataactccatgttcttttggaggagtatctgtaataactccaggaactaatacttctaatcaagtagctgtattatatcaaggagtaaattgtactgaagtaccagtagctatacatgctgatcaattaactccaacttggagagtatattctactggatctaatgtatttcaaactagagctggatgtttaataggagctgaacatgtaaataattcttatgaatgtgatataccaataggagctggaatatgtgcttcttatcaaactcaaactaattctccatctagagcctcttctgtagctagccaatctataatagcttatactatgtctttaggagctgaaaattctgtagcttattctaataattctatagctataccaactaattttactatatctgtaactactgaaatattaccagtatctatgactaaaacttctgtagattgtactatgtatatatgtggagattctactgaatgttctaatttattattacaatatggatctttttgtactcaattaaatagagctttaactggaatagctgtagaacaagataaaaatactcaagaagtatttgctcaagtaaaacaaatatataaaactccaccaataaaagattttggaggatttaatttttctcaaatattaccagatccatctaaaccatctaaaagatcttttatagaagatttattatttaataaagtaactttagctgatgctggatttataaaacaatatggagattgtttaggagatatagctgctagagatttaatatgtgctcaaaaatttaatggattaactgtattaccaccattattaactgatgaaatgatagctcaatatacttctgctttattagctggaactataacttctggatggacttttggagctggagctgctttacaaataccatttgctatgcaaatggcttatagatttaatggaataggagtaactcaaaatgtattatatgaaaatcaaaaattaatagctaatcaatttaattctgctataggaaaaatacaagattctttatcttctactgcttctgctttaggaaaattacaagatgtagtaaatcaaaatgctcaagcattaaatactttagtaaaacaattatcttctaattttggagctatatcttctgtattaaatgatatattatctagattagatccacctgaagctgaagtacaaatagatagattaataactggaagattacaatctttacaaacttatgtaactcaacaattaataagagctgctgaaataagagcttctgctaatttagctgctactaaaatgtctgaatgtgtattaggacaatctaaaagagtagatttttgtggaaaaggatatcatttaatgtcttttccacaatctgctccacatggagtagtatttttacatgtaacttatgtaccagctcaagaaaaaaattttactactgctccagctatatgtcatgatggaaaagctcattttccaagagaaggagtatttgtatctaatggaactcattggtttgtaactcaaagaaatttttatgaaccacaaataataactactgataatacttttgtatctgggaattgtgatgtagtaataggaatagtaaataatactgtatatgatccattacaaccagaattagattcttttaaagaagaattagataaatattttaaaaatcatacttctccagatgtagatttaggagatatatctggaataaatgcttctgtagtaaatatacaaaaagaaatagatagattaaatgaagtagctaaaaatttaaatgaatctttaatagatttacaagaattaggaaaatatgaacaatatataaaatggccatggtatatatggttaggatttatagctggattaatagctatagtaatggtaactataatgttatgttgtatgacttcttgttgttcttgtttaaaaggatgttgttcttgtggatcttgttgtaaatttgatgaagatgattctgaaccagtattaaaaggagtaaaattacattatacttaa

SEQ ID NO: 8 - DNA, 3816 bp, synthetic construct
  misc_feature 1..3816: note = Nucleic acid sequence of S protein from MVA-Spf-delta
  source 1..3816: mol_type = other DNA
atgtttgtatttttagtattattaccattagtatcttctcaatgtgtaaatttaagaactagaactcaattaccaccagcttatactaattcttttactagaggagtatattatccagataaagtatttagatcttctgtattacattctactcaagatttatttttaccattcttttctaatgtaacttggtttcatgctatacatgtatctggaactaatggaactaaaagatttgataatccagtattaccatttaatgatggagtatattttgcttctatagaaaaatctaatataataagaggatggatatttggaactactttagattctaaaactcaatctttattaatagtaaataatgctactaatgtagtaataaaagtatgtgaatttcaattttgtaatgatccatttttaggagtatattatcataaaaataataaatcttggatggaatctggagtatattcttctgctaataattgtacttttgaatatgtatctcaaccatttttaatggatttagaaggaaaacaaggaaattttaaaaatttaagagaatttgtatttaaaaatatagatggatattttaaaatatattctaaacatactccaataaatttagtaagagatttaccacaaggattttctgctttagaaccattagtagatttaccaataggaataaatataactagatttcaaactttattagctttacatagatcttatttaactccaggagattcttcttctggatggactgctggagctgctgcttattatgtaggatatttacaaccaagaactttcttattaaaatataatgaaaatggaactataactgatgctgtagattgtgctttagatccattatctgaaactaaatgtactttaaaatcttttactgtagaaaaaggaatatatcaaacttctaattttagagtacaaccaactgaatctatagtaagatttccaaatataactaatttatgtccatttggagaagtatttaatgctactagatttgcttctgtatatgcttggaatagaaaaagaatatctaattgtgtagctgattattctgtattatataattctgcttctttctctacttttaaatgttatggagtatctccaactaaattaaatgatttatgttttactaatgtatatgctgattcttttgtaataagaggagatgaagtaagacaaatagctccaggacaaactggaaaaatagctgattataattataaattaccagatgattttactggatgtgtaatagcttggaattctaataatttagattctaaagtaggaggaaattataattatagatatagattatttagaaaatctaatttaaaaccatttgaaagagatatatctactgaaatatatcaagctggatctaaaccatgtaatggagtagaaggatttaattgttattttccattacaatcttatggatttcaaccaactaatggagtaggatatcaaccatatagagtagtagtattatcttttgaattattacatgctccagctactgtatgtggaccaaaaaaatctactaatttagtaaaaaataaatgtgtaaattttaattttaatggattaactggaactggagtattaactgaatctaataaaaaatttttaccatttcaacaatttggaagagatatagctgatactactgatgctgtaagagatccacaaactttagaaatattagatataactccatgttcttttggaggagtatctgtaataactccaggaactaatacttctaatcaagtagctgtattatatcaaggagtaaattgtactgaagtaccagtagctatacatgctgatcaattaactccaacttggagagtatattctactggatctaatgtatttcaaactagagctggatgtttaataggagctgaacatgtaaataattcttatgaatgtgatataccaataggagctggaatatgtgcttcttatcaaactcaaactaattctagatctagagcttcttctgtagcttctcaatctataatagcttatactatgtctttaggagctgaaaattctgtagcttattctaataattctatagctataccaactaattttactatatctgtaactactgaaatattaccagtatctatgactaaaacttctgtagattgtactatgtatatatgtggagattctactgaatgttctaatttattattacaatatggatctttctgtactcaattaaatagagctttaactggaatagctgtagaacaagataaaaatactcaagaagtatttgctcaagtaaaacaaatatataaaactccaccaataaaagattttggaggatttaatttctctcaaatattaccagatccatctaaaccatctaaaagatcttttatagaagatttattatttaataaagtaactttagctgatgctggatttataaaacaatatggagattgtttaggagatatagctgctagagatttaatatgtgctcaaaaatttaatggattaactgtattaccaccattattaactgatgaaatgatagctcaatatacttctgctttattagctggaactataacttctggatggacttttggagctggagctgctttacaaataccatttgctatgcaaatggcttatagatttaatggaataggagtaactcaaaatgtattatatgaaaatcaaaaattaatagctaatcaatttaattctgctataggaaaaatacaagattctttatcttctactgcttctgctttaggaaaattacaaaatgtagtaaatcaaaatgctcaagctttaaatactttagtaaaacaattatcttctaattttggagctatatcttctgtattaaatgatatattatctagattagatccaccagaagctgaagtacaaatagatagattaataactggaagattacaatctttacaaacttatgtaactcaacaattaataagagctgctgaaataagagcttctgctaatttagctgctactaaaatgtctgaatgtgtattaggacaatctaaaagagtagatttctgtggaaaaggatatcatttaatgtcttttccacaatctgctccacatggagtagtatttttacatgtaacttatgtaccagctcaagaaaaaaattttactactgctccagctatatgtcatgatggaaaagctcattttccaagagaaggagtatttgtatctaatggaactcattggtttgtaactcaaagaaatttctatgaaccacaaataataactactgataatacttttgtatctggaaattgtgatgtagtaataggaatagtaaataatactgtatatgatccattacaaccagaattagattcttttaaagaagaattagataaatattttaaaaatcatacttctccagatgtagatttaggagatatatctggaataaatgcttctgtagtaaatatacaaaaagaaatagatagattaaatgaagtagctaaaaatttaaatgaatctttaatagatttacaagaattaggaaaatatgaacaatatataaaatggccatggtatatatggttaggatttatagctggattaatagctatagtaatggtaactataatgttatgttgtatgacttcttgttgttcttgtttaaaaggatgttgttcttgtggatcttgttgtaaatttgatgaagatgattctgaaccagtattaaaaggagtaaaattacattatacttaa

SEQ ID NO: 9 - protein, 1271 aa, synthetic construct
  REGION 1..1271: note = Amino acid sequence of S protein from MVA-Spf-delta alsorepresented in Fig. 20
MFVFLVLLPLVSSQCVNLRTRTQLPPAYTNSFTRGVYYPDKVFRSSVLHSTQDLFLPFFSNVTWFHAIHVSGTNGTKRFDNPVLPFNDGVYFASIEKSNIIRGWIFGTTLDSKTQSLLIVNNATNVVIKVCEFQFCNDPFLGVYYHKNNKSWMESGVYSSANNCTFEYVSQPFLMDLEGKQGNFKNLREFVFKNIDGYFKIYSKHTPINLVRDLPQGFSALEPLVDLPIGINITRFQTLLALHRSYLTPGDSSSGWTAGAAAYYVGYLQPRTFLLKYNENGTITDAVDCALDPLSETKCTLKSFTVEKGIYQTSNFRVQPTESIVRFPNITNLCPFGEVFNATRFASVYAWNRKRISNCVADYSVLYNSASFSTFKCYGVSPTKLNDLCFTNVYADSFVIRGDEVRQIAPGQTGKIADYNYKLPDDFTGCVIAWNSNNLDSKVGGNYNYRYRLFRKSNLKPFERDISTEIYQAGSKPCNGVEGFNCYFPLQSYGFQPTNGVGYQPYRVVVLSFELLHAPATVCGPKKSTNLVKNKCVNFNFNGLTGTGVLTESNKKFLPFQQFGRDIADTTDAVRDPQTLEILDITPCSFGGVSVITPGTNTSNQVAVLYQGVNCTEVPVAIHADQLTPTWRVYSTGSNVFQTRAGCLIGAEHVNNSYECDIPIGAGICASYQTQTNSRSRASSVASQSIIAYTMSLGAENSVAYSNNSIAIPTNFTISVTTEILPVSMTKTSVDCTMYICGDSTECSNLLLQYGSFCTQLNRALTGIAVEQDKNTQEVFAQVKQIYKTPPIKDFGGFNFSQILPDPSKPSKRSFIEDLLFNKVTLADAGFIKQYGDCLGDIAARDLICAQKFNGLTVLPPLLTDEMIAQYTSALLAGTITSGWTFGAGAALQIPFAMQMAYRFNGIGVTQNVLYENQKLIANQFNSAIGKIQDSLSSTASALGKLQNVVNQNAQALNTLVKQLSSNFGAISSVLNDILSRLDPPEAEVQIDRLITGRLQSLQTYVTQQLIRAAEIRASANLAATKMSECVLGQSKRVDFCGKGYHLMSFPQSAPHGVVFLHVTYVPAQEKNFTTAPAICHDGKAHFPREGVFVSNGTHWFVTQRNFYEPQIITTDNTFVSGNCDVVIGIVNNTVYDPLQPELDSFKEELDKYFKNHTSPDVDLGDISGINASVVNIQKEIDRLNEVAKNLNESLIDLQELGKYEQYIKWPWYIWLGFIAGLIAIVMVTIMLCCMTSCCSCLKGCCSCGSCCKFDEDDSEPVLKGVKLHYT

SEQ ID NO: 10 - DNA, 48 bp, synthetic construct
  misc_feature 1..48: note = S4800-Q5-F:
  source 1..48: mol_type = other DNA
tagattagatccacctgaagctgaagtacaaatagatagattaataac

SEQ ID NO: 11 - DNA, 31 bp, synthetic construct
  misc_feature 1..31: note = S4800-Q5-R
  source 1..31: mol_type = other DNA
gataatatatcatttaatacagaagatatag

SEQ ID NO: 12 - DNA, 31 bp, synthetic construct
  misc_feature 1..31: note = S3910-Q5-F
  source 1..31: mol_type = other DNA
gcctcttctgtagctagccaatctataatag

SEQ ID NO: 13 - DNA, 32 bp, synthetic construct
  misc_feature 1..32: note = S3910-Q5-R
  source 1..32: mol_type = other DNA
tctagatggagaattagtttgagtttgataag

SEQ ID NO: 14 - DNA, 31 bp, synthetic construct
  misc_feature 1..31: note = S3690-Q5-F
  source 1..31: mol_type = other DNA
ttatatcaaggagtaaattgtactgaagtac

SEQ ID NO: 15 - DNA, 20 bp, synthetic construct
  misc_feature 1..20: note = S3690-Q5-R
  source 1..20: mol_type = other DNA
tacagctacttgattagaag

SEQ ID NO: 16 - DNA, 38 bp, synthetic construct
  misc_feature 1..38: note = Vaccinia virus Synthetic early/late promoter
  source 1..38: mol_type = other DNA
aaaaattgaaattttatttttttttttttggaatataa

SEQ ID NO: 17 - DNA, 720 bp, synthetic construct
  misc_feature 1..720: note = GreenLantern_WR_CD
  source 1..720: mol_type = other DNA
atggtcagcaagggggaggagctcttcaccggggtcgtccccatcctcgtcgagctcgacggggacgtcaacgggcacaagttcagcgtccggggggagggggagggggacgccaccaacgggaagctcaccctcaagttcatctgcaccaccgggaagctccccgtcccctggcccaccctcgtcaccaccctcgggtacggggtcgcctgcttcgcccggtaccccgaccacatgaagcagcacgacttcttcaagagcgccatgcccgaggggtacgtccaggagcggaccatcagcttcaaggacgacgggacctacaagacgcgggccgaggtcaagttcgagggggacaccctcgtcaaccggatcgtcctcaaggggatcgacttcaaggaggacgggaacatcctcgggcacaagctcgagtacaacttcaacagccacaaggtctacatcaccgccgacaagcagaagaacgggatcaaggccaacttcaagacccggcacaacgtcgaggacgggggggtccagctcgccgaccactaccagcagaacacccccatcggggacgggcccgtcctcctccccgacaaccactacctcagccaccagagcaagctcagcaaggaccccaacgagaagcgggaccacatggtcctcaaggagcgggtcaccgccgccgggatcacccacgacatggacgagctctacaagtaa

SEQ ID NO: 18 - DNA, 720 bp, synthetic construct
  misc_feature 1..720: note = GreenLantern_WR_OP
  source 1..720: mol_type = other DNA
atggtatctaaaggagaagaattatttactggagtagtaccaatattagtagaattagatggagatgtaaatggacataaattttctgtaagaggagaaggagaaggagatgctactaatggaaaattaactttaaaatttatatgtactactggaaaattaccagtaccatggccaactttagtaactactttaggatatggagtagcttgttttgctagatatccagatcatatgaaacaacatgatttctttaaatctgctatgccagaaggatatgtacaagaaagaactatatcttttaaagatgatggaacttataaaactagagctgaagtaaaatttgaaggagatactttagtaaatagaatagtattaaaaggaatagattttaaagaagatggaaatatattaggacataaattagaatataattttaattctcataaagtatatataactgctgataaacaaaaaaatggaataaaagctaattttaaaactagacataatgtagaagatggaggagtacaattagctgatcattatcaacaaaatactccaataggagatggaccagtattattaccagataatcattatttatctcatcaatctaaattatctaaagatccaaatgaaaaaagagatcatatggtattaaaagaaagagtaactgctgctggaataactcatgatatggatgaattatataaataa

SEQ ID NO: 19 - DNA, 720 bp, synthetic construct
  misc_feature 1..720: note = >GreenLantern_HS_CD
  source 1..720: mol_type = other DNA
atggtatcgaaaggtgaagaactatttacgggtgtagtaccgatactagtagaactagatggtgatgtaaatggtcataaattttcggtacgtggtgaaggtgaaggtgatgcgacgaatggtaaactaacgctaaaatttatatgtacgacgggtaaactaccggtaccgtggccgacgctagtaacgacgctaggttatggtgtagcgtgttttgcgcgttatccggatcatatgaaacaacatgatttctttaaatcggcgatgccggaaggttatgtacaagaacgtacgatatcgtttaaagatgatggtacgtataaaacgcgtgcggaagtaaaatttgaaggtgatacgctagtaaatcgtatagtactaaaaggtatagattttaaagaagatggtaatatactaggtcataaactagaatataattttaattcgcataaagtatatataacggcggataaacaaaaaaatggtataaaagcgaattttaaaacgcgtcataatgtagaagatggtggtgtacaactagcggatcattatcaacaaaatacgccgataggtgatggtccggtactactaccggataatcattatctatcgcatcaatcgaaactatcgaaagatccgaatgaaaaacgtgatcatatggtactaaaagaacgtgtaacggcggcgggtataacgcatgatatggatgaactatataaataa

SEQ ID NO: 20 - DNA, 720 bp, synthetic construct
  misc_feature 1..720: note = >GreenLantern_HS_OP
  source 1..720: mol_type = other DNA
atggtgagcaagggcgaggagctgttcaccggcgtggtgcccatcctggtggagctggacggcgacgtgaacggccacaagttcagcgtgagaggcgagggcgagggcgacgccaccaacggcaagctgaccctgaagttcatctgcaccaccggcaagctgcccgtgccctggcccaccctggtgaccaccctgggctacggcgtggcctgcttcgccagataccccgaccacatgaagcagcacgacttcttcaagagcgccatgcccgagggctacgtgcaggagagaaccatcagcttcaaggacgacggcacctacaagaccagagccgaggtgaagttcgagggcgacaccctggtgaacagaatcgtgctgaagggcatcgacttcaaggaggacggcaacatcctgggccacaagctggagtacaacttcaacagccacaaggtgtacatcaccgccgacaagcagaagaacggcatcaaggccaacttcaagaccagacacaacgtggaggacggcggcgtgcagctggccgaccactaccagcagaacacccccatcggcgacggccccgtgctgctgcccgacaaccactacctgagccaccagagcaagctgagcaaggaccccaacgagaagagagaccacatggtgctgaaggagagagtgaccgccgccggcatcacccacgacatggacgagctgtacaagtaa

SEQ ID NO: 21 - DNA, 720 bp, synthetic construct
  misc_feature 1..720: note = >GreenLantern_VV_OP_IDT
  source 1..720: mol_type = other DNA
atggtgagtaagggtgaggagctttttactggtgtggtcccaatcctagtagagcttgacggtgatgtgaatggtcataagttttctgtgcgaggtgagggagaaggtgatgcgacgaatggtaagctaactctaaagttcatatgcactacgggtaagttgcccgtaccatggcccacacttgtgacgaccttgggttacggtgtcgcatgtttcgcccgatatccggaccatatgaaacaacatgatttcttcaaatctgcaatgccagaaggatacgttcaagaaagaacgatctcgttcaaagacgatggtacttacaaaacaagagcagaggttaagtttgagggagatacgttagtgaatcgaatcgtattaaagggtatagacttcaaagaggacggaaacatattaggtcacaaacttgagtacaacttcaactctcataaagtctacatcaccgcagataaacaaaaaaacggaattaaggcaaattttaaaacaagacataacgtcgaagatggtggtgtgcaacttgcagatcactatcaacagaacactccaataggagacggacccgtattgttgccagataatcactatttgtctcaccagtcgaagctatccaaggaccccaatgagaagcgtgaccatatggtgttgaaagagcgagtcactgctgctggaataacccatgatatggatgagctttacaagtaa

SEQ ID NO: 22 - DNA, 720 bp, synthetic construct
  misc_feature 1..720: note = >GreenLantern_HS_OP_IDT
  source 1..720: mol_type = other DNA
atggtatccaaaggcgaggagttgttcacaggggtggtccctatactggtcgaactggacggggatgtaaatggacacaaattcagtgtgagaggagaaggggagggcgacgcgaccaacggaaagctcacactcaaattcatctgtacaaccggcaaattgcctgttccgtggcccacgcttgtcacgaccctcggatacggtgtagcatgttttgcaagatatcctgaccacatgaaacaacacgacttcttcaaatctgccatgccggaggggtatgtccaggagcgcacaatcagcttcaaggacgatgggacatataaaactagagccgaagtcaagtttgagggtgacaccctcgtaaaccggatcgttctgaaaggcattgattttaaggaggacggcaatatcttgggtcataagttggagtacaattttaactctcacaaagtgtacattactgctgacaaacagaagaacgggattaaggcgaactttaagacaaggcacaacgtcgaggacggcggagtgcagctcgcggaccactatcaacaaaacactccaataggcgatggtcccgtccttcttcctgataatcattaccttagccatcaaagtaaactttctaaggacccaaatgagaagagagatcatatggtgctgaaggaaagggttaccgccgcgggaattacgcacgacatggatgagctgtataaataa

SEQ ID NO: 23 - DNA, 9304 bp, synthetic construct
  misc_feature 1..9304: note = Sequence of MVA transfer plasmid, including Sdg gene sequence (inbold).
  source 1..9304: mol_type = other DNA
gggcgaattgggcccgacgtcgcatgcgataaagtttcgaaacagcaaaaaaaatgtaaatattgtatctctaatcgtggagatgatgatagtttaagcattaatctatttattccgactattaacaagtctatatatattattatcggtttacggatgaaaaatttttggaagcctaaattcgaaatagaataatgtttttatattatacatgttctaaaagaataatcgatacagtttaagtgaaagctagagaggggtttttaaatggtcatcggtttagtcatattcgtgtctgtggcggccgccatcgtcggtgtgttgtctaacgtattggacatgtttatgtacgtagaagaaaataatgaagaggatgctagaatcaaggaggagcaagaactactgttgctatattgatacataattgaaaatctaccaacttaaatacaccgcctataaatttacaatgaaacacagattgtattctgaaggattgagtattagtaatgatttaaactcgataatcggtcaacaatctacaatggatacggatatagaaatagacgaagatgacatcatggaacttcttaatatattgactgagttaggttgtgatgtcgactttgatgaaaattttagcgatatagccgatgatattctagaatcgttgatagaacaggatgtataagtttttatgttaactaaatgtggccatttgcaccggtacctgcgggagcaaaatgtaggctggtagaaacactaccagaaaatatggattttagatccgatcatttaacaacatttgaatgttttaacgaaattatcactctagctaagaaatatatatacatagcatctttttgttgtaatcctctgagtacgactaggggagcgcttatttttgataaactaaaagaggcatctgaaaaagggattaaaataatagttttgctagatgaacgagggaaaagaaatctgggagagctacaaagtcactgcccggatataaattttataaccgttaatatagataaaaaaaataatgtgggactactactcggttgtttttgggtgtcagataatgaaagatgttatgtaggaaacgcgtcatttactggaggatctatacatacgattaaaacgttaggtgtatattctgattatcccccgctggccacagatcttcgtagaagatttgatacttttaaagcctttaatagcgcaaaaaattcatggttgaatttatgctctgcggcttgttgtctgccagttagcactgcgtatcatattaagaatcctataggtggagtgttctttactgattctccggaacacctattgggatattctagagatctagacactgatgtagttattgataaactcaagtcggctaagactagtatagatattgaacatttggccatagttcccactacacgtgtcgacggtaatagctactattggcccgacatttacaactccattatagaagcagccattaatagaggagttaagatcagacttctagttggtaattgggataagaacgacgtatattctatggcaaccgccagaagtctagacgcgttgtgtgttcaaaatgatctatctgtgaaggttttcactattcagaataatacaaaattgttgatagtcgacgacgaatatgttcatatcacttcggcaaatttcgacggaacccattaccaaaatcacggattcgtcagttttaatagtatagataaacagcttgtaagcgaggctaaaaaaatatttgagagagattgggtgagctcacattcaaagagtcttaagatataactcgagaaaaattgaaattttatttttttttttttggaatataaatgtttgtatttttagtattattaccattagtatcttctcaatgtgtaaatttaactactagaactcaattgccaccagcttatactaattcttttactagaggagtatattatccagataaagtatttagatcttctgtattacattctactcaagatttatttttaccatttttttctaatgtaacttggtttcatgctatacatgtatctggaactaatggaactaaaagatttgataatccagtattaccatttaatgatggagtatattttgcttctactgaaaaatctaatataataagaggatggatatttggaactactttagattctaaaactcaatctttattaatagtaaataatgctactaatgtagtaataaaagtatgtgaatttcaattttgtaatgatccatttttaggagtatattatcataaaaataataaatcttggatggaatctgaatttagagtatattcttctgctaataattgtacttttgaatatgtatctcaaccatttttaatggatttagaaggaaaacaaggaaattttaaaaatttaagagaatttgtatttaaaaatatagatggatattttaaaatatattctaaacatactccaataaatttagtaagagatttaccacaaggattttctgctttagaaccattagtagatttaccaataggaataaatataactagatttcaaactttattagctttacatagatcttatttaactccaggagattcttcttctggatggactgctggagctgctgcttattatgtaggatatttacaaccaagaacttttttattaaaatataatgaaaatggaactataactgatgctgtagattgtgctttagatccattatctgaaactaaatgtactttaaaatcttttactgtagaaaaaggaatatatcaaacttctaattttagagtacaaccaactgaatctatagtaagatttccaaatataactaatttatgtccatttggagaagtatttaatgctactagatttgcttctgtatatgcttggaatagaaaaagaatatctaattgtgtagctgattattctgtattatataattctgcttctttttctacttttaaatgttatggagtatctccaactaaattaaatgatttatgttttactaatgtatatgctgattcttttgtaataagaggagatgaagtaagacaaatagctccaggacaaactggaaaaatagctgattataattataaattaccagatgattttactggatgtgtaatagcttggaatagtaataatttagattctaaagtaggaggaaattataattatttatatagattatttagaaaatctaatttaaaaccatttgaaagagatatatctactgaaatatatcaagctggatctactccatgtaatggagtagaaggatttaattgttattttccattacaatcttatggatttcaaccaactaatggagtaggatatcaaccatatagagtagtagtattatcttttgaattattacatgctccagctactgtatgtggaccaaaaaaatctactaatttagtaaaaaataaatgtgtaaattttaattttaatggattaactggaactggagtattaactgaatctaataaaaaatttttaccatttcaacaatttggaagagatatagctgatactactgatgctgtaagagatccacaaactttagaaatattagatataactccatgttcttttggaggagtatctgtaataactccaggaactaatacttctaatcaagtagctgtattatatcaaggagtaaattgtactgaagtaccagtagctatacatgctgatcaattaactccaacttggagagtatattctactggatctaatgtatttcaaactagagctggatgtttaataggagctgaacatgtaaataattcttatgaatgtgatataccaataggagctggaatatgtgcttcttatcaaactcaaactaattctccaagaagagctagatctgtagctagccaatctataatagcttatactatgtctttaggagctgaaaattctgtagcttattctaataattctatagctataccaactaattttactatatctgtaactactgaaatattaccagtatctatgactaaaacttctgtagattgtactatgtatatatgtggagattctactgaatgttctaatttattattacaatatggatctttttgtactcaattaaatagagctttaactggaatagctgtagaacaagataaaaatactcaagaagtatttgctcaagtaaaacaaatatataaaactccaccaataaaagattttggaggatttaatttttctcaaatattaccagatccatctaaaccatctaaaagatcttttatagaagatttattatttaataaagtaactttagctgatgctggatttataaaacaatatggagattgtttaggagatatagctgctagagatttaatatgtgctcaaaaatttaatggattaactgtattaccaccattattaactgatgaaatgatagctcaatatacttctgctttattagctggaactataacttctggatggacttttggagctggagctgctttacaaataccatttgctatgcaaatggcttatagatttaatggaataggagtaactcaaaatgtattatatgaaaatcaaaaattaatagctaatcaatttaattctgctataggaaaaatacaagattctttatcttctactgcttctgctttaggaaaattacaagatgtagtaaatcaaaatgctcaagcattaaatactttagtaaaacaattatcttctaattttggagctatatcttctgtattaaatgatatattatctagattagataaagtagaagctgaagtacaaatagatagattaataactggaagattacaatctttacaaacttatgtaactcaacaattaataagagctgctgaaataagagcttctgctaatttagctgctactaaaatgtctgaatgtgtattaggacaatctaaaagagtagatttttgtggaaaaggatatcatttaatgtcttttccacaatctgctccacatggagtagtatttttacatgtaacttatgtaccagctcaagaaaaaaattttactactgctccagctatatgtcatgatggaaaagctcattttccaagagaaggagtatttgtatctaatggaactcattggtttgtaactcaaagaaatttttatgaaccacaaataataactactgataatacttttgtatctggaaattgtgatgtagtaataggaatagtaaataatactgtatatgatccattacaaccagaattagattcttttaaagaagaattagataaatattttaaaaatcatacttctccagatgtagatttaggagatatatctggaataaatgcttctgtagtaaatatacaaaaagaaatagatagattaaatgaagtagctaaaaatttaaatgaatctttaatagatttacaagaattaggaaaatatgaacaatatataaaatggccatggtatatatggttaggatttatagctggattaatagctatagtaatggtaactataatgttatgttgtatgacttcttgttgttcttgtttaaaaggatgttgttcttgtggatcttgttgtaaatttgatgaagatgattctgaaccagtattaaaaggagtaaaattacattatacttaattaatatcaagcttttttttattggatccggagagctcgggtatctagccacagtaaatcgttaaaaatttaaaaaatagaaacgtatagaacgccatcatgttaaacaggatacaaaccttgatgaaaacagctaacaattatgaaactattgagatattgcgtaactatttaagactgtatatcattttggcacgaaatgaagaaggtcatggtatactaatatacgatgataacatagatagtgttatgtcgatgatgaatattacaatattagaagttataggattgacgactcattgcacaaaattaagatcatcgcctccaattcctatgtctagattgtttatggacgaaatagatcatgagtcatattattctccaaaaacttcagattatccgttgatcgatattatacgaaagcgttctcacgaacagggagatatagcactggctttagaacgatacggtattgagaatacagattccatatcagaaattaatgaatggttgtcgtcaaaaggtttagcatgttatagatttgtaaaatttaacgattataggaaacagatgtatcgtaagttctctaggtgtactatagttgacagtatgataatagggcatataggtcatcattatatttggattaaaaatttagaaacatatacgcgtcccgaaattgatgtgttaccgtttgatattaaatacatatctagagatgcatagcttgagtattctatagtgtcacctaaatagcttggcgtaatcatggtcatagctgtttcctgtgtgaaattgttatccgctcacaattccacacaacatacgagccggaagcataaagtgtaaagcctggggtgcctaatgagtgagctaactcacattaattgcgttgcgctcactgcccgctttccagtcgggaaacctgtcgtgccagctgcattaatgaatcggccaacgcgcggggagaggcggtttgcgtattgggcgctcttccgcttcctcgctcactgactcgctgcgctcggtcgttcggctgcggcgagcggtatcagctcactcaaaggcggtaatacggttatccacagaatcaggggataacgcaggaaagaacatgtgagcaaaaggccagcaaaaggccaggaaccgtaaaaaggccgcgttgctggcgtttttcgataggctccgcccccctgacgagcatcacaaaaatcgacgctcaagtcagaggtggcgaaacccgacaggactataaagataccaggcgtttccccctggaagctccctcgtgcgctctcctgttccgaccctgccgcttaccggatacctgtccgcctttctcccttcgggaagcgtggcgctttctcatagctcacgctgtaggtatctcagttcggtgtaggtcgttcgctccaagctgggctgtgtgcacgaaccccccgttcagcccgaccgctgcgccttatccggtaactatcgtcttgagtccaacccggtaagacacgacttatcgccactggcagcagccactggtaacaggattagcagagcgaggtatgtaggcggtgctacagagttcttgaagtggtggcctaactacggctacactagaaggacagtatttggtatctgcgctctgctgaagccagttaccttcggaaaaagagttggtagctcttgatccggcaaacaaaccaccgctggtagcggtggtttttttgtttgcaagcagcagattacgcgcagaaaaaaaggatctcaagaagatcctttgatcttttctacggggtctgacgctcagtggaacgaaaactcacgttaagggattttggtcatgagattatcaaaaaggatcttcacctagatccttttaaattaaaaatgaagttttaaatcaatctaaagtatatatgagtaaacttggtctgacagttaccaatgcttaatcagtgaggcacctatctcagcgatctgtctatttcgttcatccatagttgcctgactccccgtcgtgtagataactacgatacgggagggcttaccatctggccccagtgctgcaatgataccgcgagacccacgctcaccggctccagatttatcagcaataaaccagccagccggaagggccgagcgcagaagtggtcctgcaactttatccgcctccatccagtctattaattgttgccgggaagctagagtaagtagttcgccagttaatagtttgcgcaacgttgttggcattgctacaggcatcgtggtgtcacgctcgtcgtttggtatggcttcattcagctccggttcccaacgatcaaggcgagttacatgatcccccatgttgtgcaaaaaagcggttagctccttcggtcctccgatcgttgtcagaagtaagttggccgcagtgttatcactcatggttatggcagcactgcataattctcttactgtcatgccatccgtaagatgcttttctgtgactggtgagtactcaaccaagtcattctgagaataccgcgcccggcgaccgagttgctcttgcccggcgtcaatacgggataatagtgtatgacatagcagaactttaaaagtgctcatcattggaaaacgttcttcggggcgaaaactctcaaggatcttaccgctgttgagatccagttcgatgtaacccactcgtgcacccaactgatcttcagcatcttttactttcaccagcgtttctgggtgagcaaaaacaggaaggcaaaatgccgcaaaaaagggaataagggcgacacggaaatgttgaatactcatactcttcctttttcaatattattgaagcatttatcagggttattgtctcatgagcggatacatatttgaatgtatttagaaaaataaacaaataggggttccgcgcacatttccccgaaaagtgccacctgtatgcggtgtgaaataccgcacagatgcgtaaggagaaaataccgcatcaggcgaaattgtaaacgttaatattttgttaaaattcgcgttaaatatttgttaaatcagctcattttttaaccaataggccgaaatcggcaaaatcccttataaatcaaaagaatagaccgagatagggttgagtgttgttccagtttggaacaagagtccactattaaagaacgtggactccaacgtcaaagggcgaaaaaccgtctatcagggcgatggcccactacgtgaaccatcacccaaatcaagttttttgcggtcgaggtgccgtaaagctctaaatcggaaccctaaagggagcccccgatttagagcttgacggggaaagccggcgaacgtggcgagaaaggaagggaagaaagcgaaaggagcgggcgctagggcgctggcaagtgtagcggtcacgctgcgcgtaaccaccacacccgccgcgcttaatgcgccgctacagggcgcgtccattcgccattcaggctgcgcaactgttgggaagggcgatcggtgcgggcctcttcgctattacgccagctggcgaaagggggatgtgctgcaaggcgattaagttgggtaacgccagggttttcccagtcacgacgttgtaaaacgacggccagtgaattgtaatacgactcactata

SEQ ID NO: 24 - DNA, 9304 bp, synthetic construct
  misc_feature 1..9304: note = Sequence of MVA transfer plasmid, including Spf gene sequence (inbold).
  source 1..9304: mol_type = other DNA
gggcgaattgggcccgacgtcgcatgcgataaagtttcgaaacagcaaaaaaaatgtaaatattgtatctctaatcgtggagatgatgatagtttaagcattaatctatttattccgactattaacaagtctatatatattattatcggtttacggatgaaaaatttttggaagcctaaattcgaaatagaataatgtttttatattatacatgttctaaaagaataatcgatacagtttaagtgaaagctagagaggggtttttaaatggtcatcggtttagtcatattcgtgtctgtggcggccgccatcgtcggtgtgttgtctaacgtattggacatgtttatgtacgtagaagaaaataatgaagaggatgctagaatcaaggaggagcaagaactactgttgctatattgatacataattgaaaatctaccaacttaaatacaccgcctataaatttacaatgaaacacagattgtattctgaaggattgagtattagtaatgatttaaactcgataatcggtcaacaatctacaatggatacggatatagaaatagacgaagatgacatcatggaacttcttaatatattgactgagttaggttgtgatgtcgactttgatgaaaattttagcgatatagccgatgatattctagaatcgttgatagaacaggatgtataagtttttatgttaactaaatgtggccatttgcaccggtacctgcgggagcaaaatgtaggctggtagaaacactaccagaaaatatggattttagatccgatcatttaacaacatttgaatgttttaacgaaattatcactctagctaagaaatatatatacatagcatctttttgttgtaatcctctgagtacgactaggggagcgcttatttttgataaactaaaagaggcatctgaaaaagggattaaaataatagttttgctagatgaacgagggaaaagaaatctgggagagctacaaagtcactgcccggatataaattttataaccgttaatatagataaaaaaaataatgtgggactactactcggttgtttttgggtgtcagataatgaaagatgttatgtaggaaacgcgtcatttactggaggatctatacatacgattaaaacgttaggtgtatattctgattatcccccgctggccacagatcttcgtagaagatttgatacttttaaagcctttaatagcgcaaaaaattcatggttgaatttatgctctgcggcttgttgtctgccagttagcactgcgtatcatattaagaatcctataggtggagtgttctttactgattctccggaacacctattgggatattctagagatctagacactgatgtagttattgataaactcaagtcggctaagactagtatagatattgaacatttggccatagttcccactacacgtgtcgacggtaatagctactattggcccgacatttacaactccattatagaagcagccattaatagaggagttaagatcagacttctagttggtaattgggataagaacgacgtatattctatggcaaccgccagaagtctagacgcgttgtgtgttcaaaatgatctatctgtgaaggttttcactattcagaataatacaaaattgttgatagtcgacgacgaatatgttcatatcacttcggcaaatttcgacggaacccattaccaaaatcacggattcgtcagttttaatagtatagataaacagcttgtaagcgaggctaaaaaaatatttgagagagattgggtgagctcacattcaaagagtcttaagatataactcgagaaaaattgaaattttatttttttttttttggaatataaatgtttgtatttttagtattattaccattagtatcttctcaatgtgtaaatttaactactagaactcaattgccaccagcttatactaattcttttactagaggagtatattatccagataaagtatttagatcttctgtattacattctactcaagatttatttttaccatttttttctaatgtaacttggtttcatgctatacatgtatctggaactaatggaactaaaagatttgataatccagtattaccatttaatgatggagtatattttgcttctactgaaaaatctaatataataagaggatggatatttggaactactttagattctaaaactcaatctttattaatagtaaataatgctactaatgtagtaataaaagtatgtgaatttcaattttgtaatgatccatttttaggagtatattatcataaaaataataaatcttggatggaatctgaatttagagtatattcttctgctaataattgtacttttgaatatgtatctcaaccatttttaatggatttagaaggaaaacaaggaaattttaaaaatttaagagaatttgtatttaaaaatatagatggatattttaaaatatattctaaacatactccaataaatttagtaagagatttaccacaaggattttctgctttagaaccattagtagatttaccaataggaataaatataactagatttcaaactttattagctttacatagatcttatttaactccaggagattcttcttctggatggactgctggagctgctgcttattatgtaggatatttacaaccaagaacttttttattaaaatataatgaaaatggaactataactgatgctgtagattgtgctttagatccattatctgaaactaaatgtactttaaaatcttttactgtagaaaaaggaatatatcaaacttctaattttagagtacaaccaactgaatctatagtaagatttccaaatataactaatttatgtccatttggagaagtatttaatgctactagatttgcttctgtatatgcttggaatagaaaaagaatatctaattgtgtagctgattattctgtattatataattctgcttctttttctacttttaaatgttatggagtatctccaactaaattaaatgatttatgttttactaatgtatatgctgattcttttgtaataagaggagatgaagtaagacaaatagctccaggacaaactggaaaaatagctgattataattataaattaccagatgattttactggatgtgtaatagcttggaatagtaataatttagattctaaagtaggaggaaattataattatttatatagattatttagaaaatctaatttaaaaccatttgaaagagatatatctactgaaatatatcaagctggatctactccatgtaatggagtagaaggatttaattgttattttccattacaatcttatggatttcaaccaactaatggagtaggatatcaaccatatagagtagtagtattatcttttgaattattacatgctccagctactgtatgtggaccaaaaaaatctactaatttagtaaaaaataaatgtgtaaattttaattttaatggattaactggaactggagtattaactgaatctaataaaaaatttttaccatttcaacaatttggaagagatatagctgatactactgatgctgtaagagatccacaaactttagaaatattagatataactccatgttcttttggaggagtatctgtaataactccaggaactaatacttctaatcaagtagctgtattatatcaaggagtaaattgtactgaagtaccagtagctatacatgctgatcaattaactccaacttggagagtatattctactggatctaatgtatttcaaactagagctggatgtttaataggagctgaacatgtaaataattcttatgaatgtgatataccaataggagctggaatatgtgcttcttatcaaactcaaactaattctccatctagagcctcttctgtagctagccaatctataatagcttatactatgtctttaggagctgaaaattctgtagcttattctaataattctatagctataccaactaattttactatatctgtaactactgaaatattaccagtatctatgactaaaacttctgtagattgtactatgtatatatgtggagattctactgaatgttctaatttattattacaatatggatctttttgtactcaattaaatagagctttaactggaatagctgtagaacaagataaaaatactcaagaagtatttgctcaagtaaaacaaatatataaaactccaccaataaaagattttggaggatttaatttttctcaaatattaccagatccatctaaaccatctaaaagatcttttatagaagatttattatttaataaagtaactttagctgatgctggatttataaaacaatatggagattgtttaggagatatagctgctagagatttaatatgtgctcaaaaatttaatggattaactgtattaccaccattattaactgatgaaatgatagctcaatatacttctgctttattagctggaactataacttctggatggacttttggagctggagctgctttacaaataccatttgctatgcaaatggcttatagatttaatggaataggagtaactcaaaatgtattatatgaaaatcaaaaattaatagctaatcaatttaattctgctataggaaaaatacaagattctttatcttctactgcttctgctttaggaaaattacaagatgtagtaaatcaaaatgctcaagcattaaatactttagtaaaacaattatcttctaattttggagctatatcttctgtattaaatgatatattatctagattagatccacctgaagctgaagtacaaatagatagattaataactggaagattacaatctttacaaacttatgtaactcaacaattaataagagctgctgaaataagagcttctgctaatttagctgctactaaaatgtctgaatgtgtattaggacaatctaaaagagtagatttttgtggaaaaggatatcatttaatgtcttttccacaatctgctccacatggagtagtatttttacatgtaacttatgtaccagctcaagaaaaaaattttactactgctccagctatatgtcatgatggaaaagctcattttccaagagaaggagtatttgtatctaatggaactcattggtttgtaactcaaagaaatttttatgaaccacaaataataactactgataatacttttgtatctgggaattgtgatgtagtaataggaatagtaaataatactgtatatgatccattacaaccagaattagattcttttaaagaagaattagataaatattttaaaaatcatacttctccagatgtagatttaggagatatatctggaataaatgcttctgtagtaaatatacaaaaagaaatagatagattaaatgaagtagctaaaaatttaaatgaatctttaatagatttacaagaattaggaaaatatgaacaatatataaaatggccatggtatatatggttaggatttatagctggattaatagctatagtaatggtaactataatgttatgttgtatgacttcttgttgttcttgtttaaaaggatgttgttcttgtggatcttgttgtaaatttgatgaagatgattctgaaccagtattaaaaggagtaaaattacattatacttaattaatatcaagcttttttttattggatccggagagctcgggtatctagccacagtaaatcgttaaaaatttaaaaaatagaaacgtatagaacgccatcatgttaaacaggatacaaaccttgatgaaaacagctaacaattatgaaactattgagatattgcgtaactatttaagactgtatatcattttggcacgaaatgaagaaggtcatggtatactaatatacgatgataacatagatagtgttatgtcgatgatgaatattacaatattagaagttataggattgacgactcattgcacaaaattaagatcatcgcctccaattcctatgtctagattgtttatggacgaaatagatcatgagtcatattattctccaaaaacttcagattatccgttgatcgatattatacgaaagcgttctcacgaacagggagatatagcactggctttagaacgatacggtattgagaatacagattccatatcagaaattaatgaatggttgtcgtcaaaaggtttagcatgttatagatttgtaaaatttaacgattataggaaacagatgtatcgtaagttctctaggtgtactatagttgacagtatgataatagggcatataggtcatcattatatttggattaaaaatttagaaacatatacgcgtcccgaaattgatgtgttaccgtttgatattaaatacatatctagagatgcatagcttgagtattctatagtgtcacctaaatagcttggcgtaatcatggtcatagctgtttcctgtgtgaaattgttatccgctcacaattccacacaacatacgagccggaagcataaagtgtaaagcctggggtgcctaatgagtgagctaactcacattaattgcgttgcgctcactgcccgctttccagtcgggaaacctgtcgtgccagctgcattaatgaatcggccaacgcgcggggagaggcggtttgcgtattgggcgctcttccgcttcctcgctcactgactcgctgcgctcggtcgttcggctgcggcgagcggtatcagctcactcaaaggcggtaatacggttatccacagaatcaggggataacgcaggaaagaacatgtgagcaaaaggccagcaaaaggccaggaaccgtaaaaaggccgcgttgctggcgtttttcgataggctccgcccccctgacgagcatcacaaaaatcgacgctcaagtcagaggtggcgaaacccgacaggactataaagataccaggcgtttccccctggaagctccctcgtgcgctctcctgttccgaccctgccgcttaccggatacctgtccgcctttctcccttcgggaagcgtggcgctttctcatagctcacgctgtaggtatctcagttcggtgtaggtcgttcgctccaagctgggctgtgtgcacgaaccccccgttcagcccgaccgctgcgccttatccggtaactatcgtcttgagtccaacccggtaagacacgacttatcgccactggcagcagccactggtaacaggattagcagagcgaggtatgtaggcggtgctacagagttcttgaagtggtggcctaactacggctacactagaaggacagtatttggtatctgcgctctgctgaagccagttaccttcggaaaaagagttggtagctcttgatccggcaaacaaaccaccgctggtagcggtggtttttttgtttgcaagcagcagattacgcgcagaaaaaaaggatctcaagaagatcctttgatcttttctacggggtctgacgctcagtggaacgaaaactcacgttaagggattttggtcatgagattatcaaaaaggatcttcacctagatccttttaaattaaaaatgaagttttaaatcaatctaaagtatatatgagtaaacttggtctgacagttaccaatgcttaatcagtgaggcacctatctcagcgatctgtctatttcgttcatccatagttgcctgactccccgtcgtgtagataactacgatacgggagggcttaccatctggccccagtgctgcaatgataccgcgagacccacgctcaccggctccagatttatcagcaataaaccagccagccggaagggccgagcgcagaagtggtcctgcaactttatccgcctccatccagtctattaattgttgccgggaagctagagtaagtagttcgccagttaatagtttgcgcaacgttgttggcattgctacaggcatcgtggtgtcacgctcgtcgtttggtatggcttcattcagctccggttcccaacgatcaaggcgagttacatgatcccccatgttgtgcaaaaaagcggttagctccttcggtcctccgatcgttgtcagaagtaagttggccgcagtgttatcactcatggttatggcagcactgcataattctcttactgtcatgccatccgtaagatgcttttctgtgactggtgagtactcaaccaagtcattctgagaataccgcgcccggcgaccgagttgctcttgcccggcgtcaatacgggataatagtgtatgacatagcagaactttaaaagtgctcatcattggaaaacgttcttcggggcgaaaactctcaaggatcttaccgctgttgagatccagttcgatgtaacccactcgtgcacccaactgatcttcagcatcttttactttcaccagcgtttctgggtgagcaaaaacaggaaggcaaaatgccgcaaaaaagggaataagggcgacacggaaatgttgaatactcatactcttcctttttcaatattattgaagcatttatcagggttattgtctcatgagcggatacatatttgaatgtatttagaaaaataaacaaataggggttccgcgcacatttccccgaaaagtgccacctgtatgcggtgtgaaataccgcacagatgcgtaaggagaaaataccgcatcaggcgaaattgtaaacgttaatattttgttaaaattcgcgttaaatatttgttaaatcagctcattttttaaccaataggccgaaatcggcaaaatcccttataaatcaaaagaatagaccgagatagggttgagtgttgttccagtttggaacaagagtccactattaaagaacgtggactccaacgtcaaagggcgaaaaaccgtctatcagggcgatggcccactacgtgaaccatcacccaaatcaagttttttgcggtcgaggtgccgtaaagctctaaatcggaaccctaaagggagcccccgatttagagcttgacggggaaagccggcgaacgtggcgagaaaggaagggaagaaagcgaaaggagcgggcgctagggcgctggcaagtgtagcggtcacgctgcgcgtaaccaccacacccgccgcgcttaatgcgccgctacagggcgcgtccattcgccattcaggctgcgcaactgttgggaagggcgatcggtgcgggcctcttcgctattacgccagctggcgaaagggggatgtgctgcaaggcgattaagttgggtaacgccagggttttcccagtcacgacgttgtaaaacgacggccagtgaattgtaatacgactcactata

SEQ ID NO: 25 - DNA, 9327 bp, synthetic construct
  misc_feature 1..9327: note = Sequence of MVA transfer plasmid, including Spfx gene sequence(in bold).
  source 1..9327: mol_type = other DNA
gggcgaattgggcccgacgtcgcatgcgataaagtttcgaaacagcaaaaaaaatgtaaatattgtatctctaatcgtggagatgatgatagtttaagcattaatctatttattccgactattaacaagtctatatatattattatcggtttacggatgaaaaatttttggaagcctaaattcgaaatagaataatgtttttatattatacatgttctaaaagaataatcgatacagtttaagtgaaagctagagaggggtttttaaatggtcatcggtttagtcatattcgtgtctgtggcggccgccatcgtcggtgtgttgtctaacgtattggacatgtttatgtacgtagaagaaaataatgaagaggatgctagaatcaaggaggagcaagaactactgttgctatattgatacataattgaaaatctaccaacttaaatacaccgcctataaatttacaatgaaacacagattgtattctgaaggattgagtattagtaatgatttaaactcgataatcggtcaacaatctacaatggatacggatatagaaatagacgaagatgacatcatggaacttcttaatatattgactgagttaggttgtgatgtcgactttgatgaaaattttagcgatatagccgatgatattctagaatcgttgatagaacaggatgtataagtttttatgttaactaaatgtggccatttgcaccggtacctgcgggagcaaaatgtaggctggtagaaacactaccagaaaatatggattttagatccgatcatttaacaacatttgaatgttttaacgaaattatcactctagctaagaaatatatatacatagcatctttttgttgtaatcctctgagtacgactaggggagcgcttatttttgataaactaaaagaggcatctgaaaaagggattaaaataatagttttgctagatgaacgagggaaaagaaatctgggagagctacaaagtcactgcccggatataaattttataaccgttaatatagataaaaaaaataatgtgggactactactcggttgtttttgggtgtcagataatgaaagatgttatgtaggaaacgcgtcatttactggaggatctatacatacgattaaaacgttaggtgtatattctgattatcccccgctggccacagatcttcgtagaagatttgatacttttaaagcctttaatagcgcaaaaaattcatggttgaatttatgctctgcggcttgttgtctgccagttagcactgcgtatcatattaagaatcctataggtggagtgttctttactgattctccggaacacctattgggatattctagagatctagacactgatgtagttattgataaactcaagtcggctaagactagtatagatattgaacatttggccatagttcccactacacgtgtcgacggtaatagctactattggcccgacatttacaactccattatagaagcagccattaatagaggagttaagatcagacttctagttggtaattgggataagaacgacgtatattctatggcaaccgccagaagtctagacgcgttgtgtgttcaaaatgatctatctgtgaaggttttcactattcagaataatacaaaattgttgatagtcgacgacgaatatgttcatatcacttcggcaaatttcgacggaacccattaccaaaatcacggattcgtcagttttaatagtatagataaacagcttgtaagcgaggctaaaaaaatatttgagagagattgggtgagctcacattcaaagagtcttaagatataactcgagaaaaattgaaattttatttttttttttttggaatataaatgtttgtatttttagtattattaccattagtatcttctcaatgtgtaaatttaactactagaactcaattgcccccggcctatactaattcgtttactcgtggtgtttactatcctgataaagtgtttcgatcgtctgtgcttcattcgactcaagatctatttttgcccttctttagtaatgttacatggttccatgctatacatgtatcgggtacaaacggtacgaagcgtttcgacaacccagtcttaccattcaatgacggagtttattttgccagtaccgagaaatcaaatatcatcagaggatggatttttggtactactttggatagtaagactcagtctctattaatcgtcaataacgcaacgaacgttgtaatcaaagtatgcgagtttcaattctgcaacgatccatttctaggtgtttactaccacaagaacaataagtcgtggatggaaagtgagttccgtgtgtactcttctgccaataactgcactttcgaatatgtttcacagccgtttttaatggacttagagggtaaacaaggtaatttcaaaaacttgagagaatttgtcttcaaaaatattgatggttatttcaaaatatattcaaagcatacgcccattaatcttgttcgagacctaccgcaaggtttttccgcattagaacccttagttgatctacccattggaatcaacattacaagattccagacattgttagctttacaccgttcgtatcttacacccggtgattcgtcatcaggatggaccgctggagctgctgcctattatgtcggttacttgcaaccgcgtacattcctattgaagtacaatgaaaatggaactattacagacgccgtggactgtgccttggatcctttatctgaaactaagtgtacattaaaatcttttacagtagaaaaaggtatttaccaaacgtccaacttccgtgtccaacccacggaatcgatagttagatttccgaatattacgaacctatgcccatttggagaagtctttaacgccacgcgttttgcctcagtttacgcttggaatcgtaagcgtattagtaactgcgtagcggattattccgtactatacaattccgcgtccttttcgactttcaaatgttacggagtgtcgcccactaaacttaacgatctttgtttcaccaacgtgtacgcagactcatttgtaatcagaggagacgaagtgcgacaaattgcgcctggtcagaccggaaaaatcgcagattacaattataaacttccggacgatttcactggttgtgtcattgcatggaattccaacaacctagacagtaaagtaggaggtaactataattacctatatagattattccgaaaatcaaatttaaaaccatttgaacgtgacatcagtacagagatataccaagcgggatctacgccgtgcaacggagtagagggatttaattgctatttcccgttacaatcgtacggattccaacccacgaacggagtaggttaccaaccgtaccgtgtcgtggtccttagttttgagttgttgcacgcacctgccaccgtgtgcggtcccaaaaagtcaacaaacttagtcaaaaacaaatgtgtcaacttcaattttaatggactaacaggaaccggagtcttgactgaatcaaacaaaaaattccttcctttccaacaattcggtcgtgatattgcggatacgacagatgcggtacgagacccgcaaacacttgagatattggatataaccccttgctcattcggtggtgtttcggtaatcacccctggaacaaacacgagtaaccaggtagccgtactttaccagggtgtgaactgtacagaggtgccagtcgcgatacatgcggatcagctaacgccaacgtggagagtatattctaccggaagtaatgtgttccaaaccagagccggatgtcttatcggtgcagaacatgtaaacaatagttacgagtgtgatatccccattggagcgggtatttgcgcaagttatcaaacccaaacaaactctccctctagagcctctagtgttgcctctcagagtatcattgcttacacgatgtcgttgggagcagaaaattctgttgcatattctaacaattcgatagcaattccaaccaatttcacgatatccgtaaccaccgagatcttgccagttagtatgactaaaacatcggttgactgcacaatgtatatatgcggtgattctactgagtgttcaaacttgcttcttcagtatggttcgttttgtactcagctaaatcgagccttgacgggaatagccgttgaacaagacaaaaatacgcaggaggtgtttgctcaagtcaaacaaatttacaagaccccacctatcaaggatttcggtggttttaacttttcccaaatattaccagacccatcaaagccaagtaagagatccttcatagaggacctattgtttaataaggtaacgttggcggacgcgggttttattaagcaatacggtgactgcttaggtgatatagctgccagagacttaatctgcgctcagaaattcaacggattaaccgttttaccaccattattgacggacgagatgatcgcgcagtatacctcggctttgctagctggtacgattacatccggttggactttcggtgccggtgcagccctacagataccatttgcgatgcaaatggcctatcgttttaatggaatcggtgtcacccagaacgtgctttacgagaaccagaagttaattgctaatcaattcaactctgcaatcggaaagattcaagactcattatctagtacagcctccgccttaggaaagttacaggacgttgtgaaccagaatgctcaggcgttaaataccttggtcaaacaactatcctcaaatttcggtgcgatatcttcagtcttgaatgatatcctaagtcgactagatccacctgaggctgaagtacagattgaccgacttatcacaggtcgtctacaaagtttgcagacgtatgtgacccaacagctaataagagcggctgagatacgtgcttctgccaatttagcagctacaaaaatgtcagagtgtgtgctaggacaatcgaaacgagttgacttctgtggaaagggttaccacttgatgtcattcccccaaagtgcgcctcatggtgtggttttcttgcatgtaacgtacgtacccgcgcaagaaaagaattttactaccgccccggccatttgtcatgacggaaaagctcattttccgcgtgaaggtgtattcgtatccaacggtacgcactggtttgtgacccaaagaaacttttatgaaccgcagattataacgaccgacaatacgttcgtgtctggaaattgcgacgttgtaattggaatcgtaaacaatacagtttacgacccattgcaacccgagctagatagttttaaggaagaacttgacaagtattttaagaaccacacgtcaccggacgtcgacttgggagatatttcgggaattaacgctagtgttgtgaatatccagaaagaaatagatcgactaaatgaagtggccaagaaccttaacgagtccctaattgacttacaggaattgggtaagtatgaacaatacataaaatggccatggtatatatggttaggatttatagctggattaatagctatagtaatggttactatcatgttatgctgcatgacctcctgctgttcatgtttaaaaggatgttgctcctgcggttcgtgttgtaagttcgatgaagatgactccgaacctgtcttgaagggagtgaaattgcattacacttaattaatatcaagctttaaccatggaggcctaaataaataatttttatggatccggagagctcgggtatctagccacagtaaatcgttaaaaatttaaaaaatagaaacgtatagaacgccatcatgttaaacaggatacaaaccttgatgaaaacagctaacaattatgaaactattgagatattgcgtaactatttaagactgtatatcattttggcacgaaatgaagaaggtcatggtatactaatatacgatgataacatagatagtgttatgtcgatgatgaatattacaatattagaagttataggattgacgactcattgcacaaaattaagatcatcgcctccaattcctatgtctagattgtttatggacgaaatagatcatgagtcatattattctccaaaaacttcagattatccgttgatcgatattatacgaaagcgttctcacgaacagggagatatagcactggctttagaacgatacggtattgagaatacagattccatatcagaaattaatgaatggttgtcgtcaaaaggtttagcatgttatagatttgtaaaatttaacgattataggaaacagatgtatcgtaagttctctaggtgtactatagttgacagtatgataatagggcatataggtcatcattatatttggattaaaaatttagaaacatatacgcgtcccgaaattgatgtgttaccgtttgatattaaatacatatctagagatgcatagcttgagtattctatagtgtcacctaaatagcttggcgtaatcatggtcatagctgtttcctgtgtgaaattgttatccgctcacaattccacacaacatacgagccggaagcataaagtgtaaagcctggggtgcctaatgagtgagctaactcacattaattgcgttgcgctcactgcccgctttccagtcgggaaacctgtcgtgccagctgcattaatgaatcggccaacgcgcggggagaggcggtttgcgtattgggcgctcttccgcttcctcgctcactgactcgctgcgctcggtcgttcggctgcggcgagcggtatcagctcactcaaaggcggtaatacggttatccacagaatcaggggataacgcaggaaagaacatgtgagcaaaaggccagcaaaaggccaggaaccgtaaaaaggccgcgttgctggcgtttttcgataggctccgcccccctgacgagcatcacaaaaatcgacgctcaagtcagaggtggcgaaacccgacaggactataaagataccaggcgtttccccctggaagctccctcgtgcgctctcctgttccgaccctgccgcttaccggatacctgtccgcctttctcccttcgggaagcgtggcgctttctcatagctcacgctgtaggtatctcagttcggtgtaggtcgttcgctccaagctgggctgtgtgcacgaaccccccgttcagcccgaccgctgcgccttatccggtaactatcgtcttgagtccaacccggtaagacacgacttatcgccactggcagcagccactggtaacaggattagcagagcgaggtatgtaggcggtgctacagagttcttgaagtggtggcctaactacggctacactagaaggacagtatttggtatctgcgctctgctgaagccagttaccttcggaaaaagagttggtagctcttgatccggcaaacaaaccaccgctggtagcggtggtttttttgtttgcaagcagcagattacgcgcagaaaaaaaggatctcaagaagatcctttgatcttttctacggggtctgacgctcagtggaacgaaaactcacgttaagggattttggtcatgagattatcaaaaaggatcttcacctagatccttttaaattaaaaatgaagttttaaatcaatctaaagtatatatgagtaaacttggtctgacagttaccaatgcttaatcagtgaggcacctatctcagcgatctgtctatttcgttcatccatagttgcctgactccccgtcgtgtagataactacgatacgggagggcttaccatctggccccagtgctgcaatgataccgcgagacccacgctcaccggctccagatttatcagcaataaaccagccagccggaagggccgagcgcagaagtggtcctgcaactttatccgcctccatccagtctattaattgttgccgggaagctagagtaagtagttcgccagttaatagtttgcgcaacgttgttggcattgctacaggcatcgtggtgtcacgctcgtcgtttggtatggcttcattcagctccggttcccaacgatcaaggcgagttacatgatcccccatgttgtgcaaaaaagcggttagctccttcggtcctccgatcgttgtcagaagtaagttggccgcagtgttatcactcatggttatggcagcactgcataattctcttactgtcatgccatccgtaagatgcttttctgtgactggtgagtactcaaccaagtcattctgagaataccgcgcccggcgaccgagttgctcttgcccggcgtcaatacgggataatagtgtatgacatagcagaactttaaaagtgctcatcattggaaaacgttcttcggggcgaaaactctcaaggatcttaccgctgttgagatccagttcgatgtaacccactcgtgcacccaactgatcttcagcatcttttactttcaccagcgtttctgggtgagcaaaaacaggaaggcaaaatgccgcaaaaaagggaataagggcgacacggaaatgttgaatactcatactcttcctttttcaatattattgaagcatttatcagggttattgtctcatgagcggatacatatttgaatgtatttagaaaaataaacaaataggggttccgcgcacatttccccgaaaagtgccacctgtatgcggtgtgaaataccgcacagatgcgtaaggagaaaataccgcatcaggcgaaattgtaaacgttaatattttgttaaaattcgcgttaaatatttgttaaatcagctcattttttaaccaataggccgaaatcggcaaaatcccttataaatcaaaagaatagaccgagatagggttgagtgttgttccagtttggaacaagagtccactattaaagaacgtggactccaacgtcaaagggcgaaaaaccgtctatcagggcgatggcccactacgtgaaccatcacccaaatcaagttttttgcggtcgaggtgccgtaaagctctaaatcggaaccctaaagggagcccccgatttagagcttgacggggaaagccggcgaacgtggcgagaaaggaagggaagaaagcgaaaggagcgggcgctagggcgctggcaagtgtagcggtcacgctgcgcgtaaccaccacacccgccgcgcttaatgcgccgctacagggcgcgtccattcgccattcaggctgcgcaactgttgggaagggcgatcggtgcgggcctcttcgctattacgccagctggcgaaagggggatgtgctgcaaggcgattaagttgggtaacgccagggttttcccagtcacgacgttgtaaaacgacggccagtgaattgtaatacgactcactata

SEQ ID NO: 26 - DNA, 9299 bp, synthetic construct
  misc_feature 1..9299: note = Sequence of MVA transfer plasmid, including Spf-o (omicron) genesequence (in bold).
  source 1..9299: mol_type = other DNA
gggcgaattgggcccgacgtcgcatgcgataaagtttcgaaacagcaaaaaaaatgtaaatattgtatctctaatcgtggagatgatgatagtttaagcattaatctatttattccgactattaacaagtctatatatattattatcggtttacggatgaaaaatttttggaagcctaaattcgaaatagaataatgtttttatattatacatgttctaaaagaataatcgatacagtttaagtgaaagctagagaggggtttttaaatggtcatcggtttagtcatattcgtgtctgtggcggccgccatcgtcggtgtgttgtctaacgtattggacatgtttatgtacgtagaagaaaataatgaagaggatgctagaatcaaggaggagcaagaactactgttgctatattgatacataattgaaaatctaccaacttaaatacaccgcctataaatttacaatgaaacacagattgtattctgaaggattgagtattagtaatgatttaaactcgataatcggtcaacaatctacaatggatacggatatagaaatagacgaagatgacatcatggaacttcttaatatattgactgagttaggttgtgatgtcgactttgatgaaaattttagcgatatagccgatgatattctagaatcgttgatagaacaggatgtataagtttttatgttaactaaatgtggccatttgcaccggtacctgcgggagcaaaatgtaggctggtagaaacactaccagaaaatatggattttagatccgatcatttaacaacatttgaatgttttaacgaaattatcactctagctaagaaatatatatacatagcatctttttgttgtaatcctctgagtacgactaggggagcgcttatttttgataaactaaaagaggcatctgaaaaagggattaaaataatagttttgctagatgaacgagggaaaagaaatctgggagagctacaaagtcactgcccggatataaattttataaccgttaatatagataaaaaaaataatgtgggactactactcggttgtttttgggtgtcagataatgaaagatgttatgtaggaaacgcgtcatttactggaggatctatacatacgattaaaacgttaggtgtatattctgattatcccccgctggccacagatcttcgtagaagatttgatacttttaaagcctttaatagcgcaaaaaattcatggttgaatttatgctctgcggcttgttgtctgccagttagcactgcgtatcatattaagaatcctataggtggagtgttctttactgattctccggaacacctattgggatattctagagatctagacactgatgtagttattgataaactcaagtcggctaagactagtatagatattgaacatttggccatagttcccactacacgtgtcgacggtaatagctactattggcccgacatttacaactccattatagaagcagccattaatagaggagttaagatcagacttctagttggtaattgggataagaacgacgtatattctatggcaaccgccagaagtctagacgcgttgtgtgttcaaaatgatctatctgtgaaggttttcactattcagaataatacaaaattgttgatagtcgacgacgaatatgttcatatcacttcggcaaatttcgacggaacccattaccaaaatcacggattcgtcagttttaatagtatagataaacagcttgtaagcgaggctaaaaaaatatttgagagagattgggtgagctcacattcaaagagtcttaagatataactcgagaaaaattgaaattttatttttttttttttggaatataaatgtttgtatttttagtattattaccattagtatcttctcaatgtgtaaatttaataactagaactcaatcttatactaattcttttactagaggagtatattatccagataaagtatttagatcttctgtattacattctactcaagatttatttttaccattcttctctaatgtaacttggtttcatgctatacatgtatctggaactaatggaactaaaagatttgataatccagtattaccatttaatgatggagtatattttgcttctactgaaaaatctaatataataagaggatggatatttggaactactttagattctaaaactcaatctttattaatagtaaataatgctactaatgtagtaataaaagtatgtgaatttcaattttgtaatgatccatttttagatgtatattatcataaaaataataaatcttggatggaatctgaatttagagtatattcttctgctaataattgtacttttgaatatgtatctcaaccatttttaatggatttagaaggaaaacaaggaaattttaaaaatttaagagaatttgtatttaaaaatatagatggatattttaaaatatattctaaacatactccaataaatttaggaagagatttaccacaaggattttctgctttagaaccattagtagatttaccaataggaataaatataactagatttcaaactttattagctttacatagatcttatttaactccaggagattcttcttctggatggactgctggagctgctgcttattatgtaggatatttacaaccaagaactttcttattaaaatataatgaaaatggaactataactgatgctgtagattgtgctttagatccattatctgaaactaaatgtactttaaaatcttttactgtagaaaaaggaatatatcaaacttctaattttagagtacaaccaactgaatctatagtaagatttccaaatataactaatttatgtccatttgatgaagtatttaatgctactagatttgcttctgtatatgcttggaatagaaaaagaatatctaattgtgtagctgattattctgtattatataattttgctccattttttgcttttaaatgttatggagtatctccaactaaattaaatgatttatgttttactaatgtatatgctgattcttttgtaataagaggaaatgaagtatctcaaatagctccaggacaaactggaaatatagctgattataattataaattaccagatgattttactggatgtgtaatagcttggaattctaataaattagattctaaagtaggaggaaattataattatttatatagattatttagaaaatctaatttaaaaccatttgaaagagatatatctactgaaatatatcaagctggaaataaaccatgtaatggagtagctggatttaattgttattttccattaagatcttatggatttagaccaacttatggagtaggacatcaaccatatagagtagtagtattatcttttgaattattacatgctccagctactgtatgtggaccaaaaaaatctactaatttagtaaaaaataaatgtgtaaattttaattttaatggattaactggaactggagtattaactgaatctaataaaaaatttttaccatttcaacaatttggaagagatatagctgatactactgatgctgtaagagatccacaaactttagaaatattagatataactccatgttcttttggaggagtatctgtaataactccaggaactaatacttctaatcaagtagctgtattatatcaaggagtaaattgtactgaagtaccagtagctatacatgctgatcaattaactccaacttggagagtatattctactggatctaatgtatttcaaactagagctggatgtttaataggagctgaatatgtaaataattcttatgaatgtgatataccaataggagctggaatatgtgcttcttatcaaactcaaactaaatctcatagtagagctagttctgtagcttctcaatctataatagcttatactatgtctttaggagctgaaaattctgtagcttattctaataattctatagctataccaactaattttactatatctgtaactactgaaatattaccagtatctatgactaaaacttctgtagattgtactatgtatatatgtggagattctactgaatgttctaatttattattacaatatggatctttctgtactcaattaaaaagagctttaactggaatagctgtagaacaagataaaaatactcaagaagtatttgctcaagtaaaacaaatatataaaactccaccaataaaatattttggaggatttaatttctctcaaatattaccagatccatctaaaccatctaaaagatcttttatagaagatttattatttaataaagtaactttagctgatgctggatttataaaacaatatggagattgtttaggagatatagctgctagagatttaatatgtgctcaaaaatttaatggattaactgtattaccaccattattaactgatgaaatgatagctcaatatacttctgctttattagctggaactataacttctggatggacttttggagctggagctgctttacaaataccatttgctatgcaaatggcttatagatttaatggaataggagtaactcaaaatgtattatatgaaaatcaaaaattaatagctaatcaatttaattctgctataggaaaaatacaagattctttatcttctactgcttctgctttaggaaaattacaagatgtagtaaatcataatgctcaagctttaaatactttagtaaaacaattatcttctaaatttggagctatatcttctgtattaaatgatatattatctagattagatccaccagaagctgaagtacaaatagatagattaataactggaagattacaatctttacaaacttatgtaactcaacaattaataagagctgctgaaataagagcttctgctaatttagctgctactaaaatgtctgaatgtgtattaggacaatctaaaagagtagatttctgtggaaaaggatatcatttaatgtcttttccacaatctgctccacatggagtagtatttttacatgtaacttatgtaccagctcaagaaaaaaattttactactgctccagctatatgtcatgatggaaaagctcattttccaagagaaggagtatttgtatctaatggaactcattggtttgtaactcaaagaaatttctatgaaccacaaataataactactgataatacttttgtatctggaaattgtgatgtagtaataggaatagtaaataatactgtatatgatccattacaaccagaattagattcttttaaagaagaattagataaatattttaaaaatcatacttctccagatgtagatttaggagatatatctggaataaatgcttctgtagtaaatatacaaaaagaaatagatagattaaatgaagtagctaaaaatttaaatgaatctttaatagatttacaagaattaggaaaatatgaacaatatataaaatggccatggtatatatggttaggatttatagctggattaatagctatagtaatggtaactataatgttatgttgtatgacttcttgttgttcttgtttaaaaggatgttgttcttgtggatcttgttgtaaatttgatgaagatgattctgaaccagtattaaaaggagtaaaattacattatacttaattaattaatatcaagcttttttttattggatccggagagctcgggtatctagccacagtaaatcgttaaaaatttaaaaaatagaaacgtatagaacgccatcatgttaaacaggatacaaaccttgatgaaaacagctaacaattatgaaactattgagatattgcgtaactatttaagactgtatatcattttggcacgaaatgaagaaggtcatggtatactaatatacgatgataacatagatagtgttatgtcgatgatgaatattacaatattagaagttataggattgacgactcattgcacaaaattaagatcatcgcctccaattcctatgtctagattgtttatggacgaaatagatcatgagtcatattattctccaaaaacttcagattatccgttgatcgatattatacgaaagcgttctcacgaacagggagatatagcactggctttagaacgatacggtattgagaatacagattccatatcagaaattaatgaatggttgtcgtcaaaaggtttagcatgttatagatttgtaaaatttaacgattataggaaacagatgtatcgtaagttctctaggtgtactatagttgacagtatgataatagggcatataggtcatcattatatttggattaaaaatttagaaacatatacgcgtcccgaaattgatgtgttaccgtttgatattaaatacatatctagagatgcatagcttgagtattctatagtgtcacctaaatagcttggcgtaatcatggtcatagctgtttcctgtgtgaaattgttatccgctcacaattccacacaacatacgagccggaagcataaagtgtaaagcctggggtgcctaatgagtgagctaactcacattaattgcgttgcgctcactgcccgctttccagtcgggaaacctgtcgtgccagctgcattaatgaatcggccaacgcgcggggagaggcggtttgcgtattgggcgctcttccgcttcctcgctcactgactcgctgcgctcggtcgttcggctgcggcgagcggtatcagctcactcaaaggcggtaatacggttatccacagaatcaggggataacgcaggaaagaacatgtgagcaaaaggccagcaaaaggccaggaaccgtaaaaaggccgcgttgctggcgtttttcgataggctccgcccccctgacgagcatcacaaaaatcgacgctcaagtcagaggtggcgaaacccgacaggactataaagataccaggcgtttccccctggaagctccctcgtgcgctctcctgttccgaccctgccgcttaccggatacctgtccgcctttctcccttcgggaagcgtggcgctttctcatagctcacgctgtaggtatctcagttcggtgtaggtcgttcgctccaagctgggctgtgtgcacgaaccccccgttcagcccgaccgctgcgccttatccggtaactatcgtcttgagtccaacccggtaagacacgacttatcgccactggcagcagccactggtaacaggattagcagagcgaggtatgtaggcggtgctacagagttcttgaagtggtggcctaactacggctacactagaaggacagtatttggtatctgcgctctgctgaagccagttaccttcggaaaaagagttggtagctcttgatccggcaaacaaaccaccgctggtagcggtggtttttttgtttgcaagcagcagattacgcgcagaaaaaaaggatctcaagaagatcctttgatcttttctacggggtctgacgctcagtggaacgaaaactcacgttaagggattttggtcatgagattatcaaaaaggatcttcacctagatccttttaaattaaaaatgaagttttaaatcaatctaaagtatatatgagtaaacttggtctgacagttaccaatgcttaatcagtgaggcacctatctcagcgatctgtctatttcgttcatccatagttgcctgactccccgtcgtgtagataactacgatacgggagggcttaccatctggccccagtgctgcaatgataccgcgagacccacgctcaccggctccagatttatcagcaataaaccagccagccggaagggccgagcgcagaagtggtcctgcaactttatccgcctccatccagtctattaattgttgccgggaagctagagtaagtagttcgccagttaatagtttgcgcaacgttgttggcattgctacaggcatcgtggtgtcacgctcgtcgtttggtatggcttcattcagctccggttcccaacgatcaaggcgagttacatgatcccccatgttgtgcaaaaaagcggttagctccttcggtcctccgatcgttgtcagaagtaagttggccgcagtgttatcactcatggttatggcagcactgcataattctcttactgtcatgccatccgtaagatgcttttctgtgactggtgagtactcaaccaagtcattctgagaataccgcgcccggcgaccgagttgctcttgcccggcgtcaatacgggataatagtgtatgacatagcagaactttaaaagtgctcatcattggaaaacgttcttcggggcgaaaactctcaaggatcttaccgctgttgagatccagttcgatgtaacccactcgtgcacccaactgatcttcagcatcttttactttcaccagcgtttctgggtgagcaaaaacaggaaggcaaaatgccgcaaaaaagggaataagggcgacacggaaatgttgaatactcatactcttcctttttcaatattattgaagcatttatcagggttattgtctcatgagcggatacatatttgaatgtatttagaaaaataaacaaataggggttccgcgcacatttccccgaaaagtgccacctgtatgcggtgtgaaataccgcacagatgcgtaaggagaaaataccgcatcaggcgaaattgtaaacgttaatattttgttaaaattcgcgttaaatatttgttaaatcagctcattttttaaccaataggccgaaatcggcaaaatcccttataaatcaaaagaatagaccgagatagggttgagtgttgttccagtttggaacaagagtccactattaaagaacgtggactccaacgtcaaagggcgaaaaaccgtctatcagggcgatggcccactacgtgaaccatcacccaaatcaagttttttgcggtcgaggtgccgtaaagctctaaatcggaaccctaaagggagcccccgatttagagcttgacggggaaagccggcgaacgtggcgagaaaggaagggaagaaagcgaaaggagcgggcgctagggcgctggcaagtgtagcggtcacgctgcgcgtaaccaccacacccgccgcgcttaatgcgccgctacagggcgcgtccattcgccattcaggctgcgcaactgttgggaagggcgatcggtgcgggcctcttcgctattacgccagctggcgaaagggggatgtgctgcaaggcgattaagttgggtaacgccagggttttcccagtcacgacgttgtaaaacgacggccagtgaattgtaatacgactcactata

SEQ ID NO: 27 - DNA, 3813 bp, synthetic construct
  misc_feature 1..3813: note = Nucleic acid sequence of S protein from MVA-Spf-o (omicron)
  source 1..3813: mol_type = other DNA
atgtttgtatttttagtattattaccattagtatcttctcaatgtgtaaatttaataactagaactcaatcttatactaattcttttactagaggagtatattatccagataaagtatttagatcttctgtattacattctactcaagatttatttttaccattcttctctaatgtaacttggtttcatgctatacatgtatctggaactaatggaactaaaagatttgataatccagtattaccatttaatgatggagtatattttgcttctactgaaaaatctaatataataagaggatggatatttggaactactttagattctaaaactcaatctttattaatagtaaataatgctactaatgtagtaataaaagtatgtgaatttcaattttgtaatgatccatttttagatgtatattatcataaaaataataaatcttggatggaatctgaatttagagtatattcttctgctaataattgtacttttgaatatgtatctcaaccatttttaatggatttagaaggaaaacaaggaaattttaaaaatttaagagaatttgtatttaaaaatatagatggatattttaaaatatattctaaacatactccaataaatttaggaagagatttaccacaaggattttctgctttagaaccattagtagatttaccaataggaataaatataactagatttcaaactttattagctttacatagatcttatttaactccaggagattcttcttctggatggactgctggagctgctgcttattatgtaggatatttacaaccaagaactttcttattaaaatataatgaaaatggaactataactgatgctgtagattgtgctttagatccattatctgaaactaaatgtactttaaaatcttttactgtagaaaaaggaatatatcaaacttctaattttagagtacaaccaactgaatctatagtaagatttccaaatataactaatttatgtccatttgatgaagtatttaatgctactagatttgcttctgtatatgcttggaatagaaaaagaatatctaattgtgtagctgattattctgtattatataattttgctccattttttgcttttaaatgttatggagtatctccaactaaattaaatgatttatgttttactaatgtatatgctgattcttttgtaataagaggaaatgaagtatctcaaatagctccaggacaaactggaaatatagctgattataattataaattaccagatgattttactggatgtgtaatagcttggaattctaataaattagattctaaagtaggaggaaattataattatttatatagattatttagaaaatctaatttaaaaccatttgaaagagatatatctactgaaatatatcaagctggaaataaaccatgtaatggagtagctggatttaattgttattttccattaagatcttatggatttagaccaacttatggagtaggacatcaaccatatagagtagtagtattatcttttgaattattacatgctccagctactgtatgtggaccaaaaaaatctactaatttagtaaaaaataaatgtgtaaattttaattttaatggattaactggaactggagtattaactgaatctaataaaaaatttttaccatttcaacaatttggaagagatatagctgatactactgatgctgtaagagatccacaaactttagaaatattagatataactccatgttcttttggaggagtatctgtaataactccaggaactaatacttctaatcaagtagctgtattatatcaaggagtaaattgtactgaagtaccagtagctatacatgctgatcaattaactccaacttggagagtatattctactggatctaatgtatttcaaactagagctggatgtttaataggagctgaatatgtaaataattcttatgaatgtgatataccaataggagctggaatatgtgcttcttatcaaactcaaactaaatctcatagtagagctagttctgtagcttctcaatctataatagcttatactatgtctttaggagctgaaaattctgtagcttattctaataattctatagctataccaactaattttactatatctgtaactactgaaatattaccagtatctatgactaaaacttctgtagattgtactatgtatatatgtggagattctactgaatgttctaatttattattacaatatggatctttctgtactcaattaaaaagagctttaactggaatagctgtagaacaagataaaaatactcaagaagtatttgctcaagtaaaacaaatatataaaactccaccaataaaatattttggaggatttaatttctctcaaatattaccagatccatctaaaccatctaaaagatcttttatagaagatttattatttaataaagtaactttagctgatgctggatttataaaacaatatggagattgtttaggagatatagctgctagagatttaatatgtgctcaaaaatttaatggattaactgtattaccaccattattaactgatgaaatgatagctcaatatacttctgctttattagctggaactataacttctggatggacttttggagctggagctgctttacaaataccatttgctatgcaaatggcttatagatttaatggaataggagtaactcaaaatgtattatatgaaaatcaaaaattaatagctaatcaatttaattctgctataggaaaaatacaagattctttatcttctactgcttctgctttaggaaaattacaagatgtagtaaatcataatgctcaagctttaaatactttagtaaaacaattatcttctaaatttggagctatatcttctgtattaaatgatatattatctagattagatccaccagaagctgaagtacaaatagatagattaataactggaagattacaatctttacaaacttatgtaactcaacaattaataagagctgctgaaataagagcttctgctaatttagctgctactaaaatgtctgaatgtgtattaggacaatctaaaagagtagatttctgtggaaaaggatatcatttaatgtcttttccacaatctgctccacatggagtagtatttttacatgtaacttatgtaccagctcaagaaaaaaattttactactgctccagctatatgtcatgatggaaaagctcattttccaagagaaggagtatttgtatctaatggaactcattggtttgtaactcaaagaaatttctatgaaccacaaataataactactgataatacttttgtatctggaaattgtgatgtagtaataggaatagtaaataatactgtatatgatccattacaaccagaattagattcttttaaagaagaattagataaatattttaaaaatcatacttctccagatgtagatttaggagatatatctggaataaatgcttctgtagtaaatatacaaaaagaaatagatagattaaatgaagtagctaaaaatttaaatgaatctttaatagatttacaagaattaggaaaatatgaacaatatataaaatggccatggtatatatggttaggatttatagctggattaatagctatagtaatggtaactataatgttatgttgtatgacttcttgttgttcttgtttaaaaggatgttgttcttgtggatcttgttgtaaatttgatgaagatgattctgaaccagtattaaaaggagtaaaattacattatacttaa

SEQ ID NO: 28 - protein, 1270 aa, synthetic construct
  REGION 1..1270: note = Amino acid sequence of S protein from MVA-Spf-o (omicron) alsorepresented in Fig. 20
MFVFLVLLPLVSSQCVNLITRTQSYTNSFTRGVYYPDKVFRSSVLHSTQDLFLPFFSNVTWFHAIHVSGTNGTKRFDNPVLPFNDGVYFASTEKSNIIRGWIFGTTLDSKTQSLLIVNNATNVVIKVCEFQFCNDPFLDVYYHKNNKSWMESEFRVYSSANNCTFEYVSQPFLMDLEGKQGNFKNLREFVFKNIDGYFKIYSKHTPINLGRDLPQGFSALEPLVDLPIGINITRFQTLLALHRSYLTPGDSSSGWTAGAAAYYVGYLQPRTFLLKYNENGTITDAVDCALDPLSETKCTLKSFTVEKGIYQTSNFRVQPTESIVRFPNITNLCPFDEVFNATRFASVYAWNRKRISNCVADYSVLYNFAPFFAFKCYGVSPTKLNDLCFTNVYADSFVIRGNEVSQIAPGQTGNIADYNYKLPDDFTGCVIAWNSNKLDSKVGGNYNYLYRLFRKSNLKPFERDISTEIYQAGNKPCNGVAGFNCYFPLRSYGFRPTYGVGHQPYRVVVLSFELLHAPATVCGPKKSTNLVKNKCVNFNFNGLTGTGVLTESNKKFLPFQQFGRDIADTTDAVRDPQTLEILDITPCSFGGVSVITPGTNTSNQVAVLYQGVNCTEVPVAIHADQLTPTWRVYSTGSNVFQTRAGCLIGAEYVNNSYECDIPIGAGICASYQTQTKSHSRASSVASQSIIAYTMSLGAENSVAYSNNSIAIPTNFTISVTTEILPVSMTKTSVDCTMYICGDSTECSNLLLQYGSFCTQLKRALTGIAVEQDKNTQEVFAQVKQIYKTPPIKYFGGFNFSQILPDPSKPSKRSFIEDLLFNKVTLADAGFIKQYGDCLGDIAARDLICAQKFNGLTVLPPLLTDEMIAQYTSALLAGTITSGWTFGAGAALQIPFAMQMAYRFNGIGVTQNVLYENQKLIANQFNSAIGKIQDSLSSTASALGKLQDVVNHNAQALNTLVKQLSSKFGAISSVLNDILSRLDPPEAEVQIDRLITGRLQSLQTYVTQQLIRAAEIRASANLAATKMSECVLGQSKRVDFCGKGYHLMSFPQSAPHGVVFLHVTYVPAQEKNFTTAPAICHDGKAHFPREGVFVSNGTHWFVTQRNFYEPQIITTDNTFVSGNCDVVIGIVNNTVYDPLQPELDSFKEELDKYFKNHTSPDVDLGDISGINASVVNIQKEIDRLNEVAKNLNESLIDLQELGKYEQYIKWPWYIWLGFIAGLIAIVMVTIMLCCMTSCCSCLKGCCSCGSCCKFDEDDSEPVLKGVKLHYT